European Patent Application EP 4 218 932 A2, published August 2, 2023. Title: Multispecific anti-TCR delta variable 1 antibodies. Applicant: GammaDelta Therapeutics Limited. Application EP. The sequence listing filed with the application follows.

SEQUENCE LISTING (176 sequences)

SEQ ID NO: 1 - protein, 209 aa, Homo sapiens
  REGION 1..209: note = Variable delta 1 (V delta 1) chain of a gamma delta T cell receptor (TCR) (human)
AQKVTQAQSSVSMPVRKAVTLNCLYETSWWSYYIFWYKQLPSKEMIFLIRQGSDEQNAKSGRYSVNFKKAAKSVALTISALQLEDSAKYFCALGESLTRADKLIFGKGTRVTVEPNIQNPDPAVYQLRDSKSSDKSVCLFTDFDSQTNVSQSKDSDVYITDKTVLDMRSMDFKSNSAVAWSNKSDFACANAFNNSIIPEDTFFPSPESS

SEQ ID NO: 2 - protein, 9 aa, Homo sapiens
  REGION 1..9: note = E07 Heavy CDR3
VDYADAFDI

SEQ ID NO: 3 - protein, 9 aa, Homo sapiens
  REGION 1..9: note = C08 Heavy CDR3
PIELGAFDI

SEQ ID NO: 4 - protein, 8 aa, Homo sapiens
  REGION 1..8: note = G04 Heavy CDR3
TWSGYVDV

SEQ ID NO: 5 - protein, 9 aa, Homo sapiens
  REGION 1..9: note = B07 Heavy CDR3
ENYLNAFDI

SEQ ID NO: 6 - protein, 8 aa, Homo sapiens
  REGION 1..8: note = C05 Heavy CDR3
DSGVAFDI

SEQ ID NO: 7 - protein, 10 aa, Homo sapiens
  REGION 1..10: note = E01 Heavy CDR3
HQVDTRTADY

SEQ ID NO: 8 - protein, 8 aa, Homo sapiens
  REGION 1..8: note = E04 Heavy CDR3
SWNDAFDI

SEQ ID NO: 9 - protein, 8 aa, Homo sapiens
  REGION 1..8: note = F07 Heavy CDR3
DYYYSMDV

SEQ ID NO: 10 - protein, 9 aa, Homo sapiens
  REGION 1..9: note = G06 Heavy CDR3
HSWNDAFDV

SEQ ID NO: 11 - protein, 8 aa, Homo sapiens
  REGION 1..8: note = G09 Heavy CDR3
DYYYSMDV

SEQ ID NO: 12 - protein, 9 aa, Homo sapiens
  REGION 1..9: note = B09 Heavy CDR3
HSWSDAFDI

SEQ ID NO: 13 - protein, 9 aa, Homo sapiens
  REGION 1..9: note = G10 Heavy CDR3
HSWNDAFDI

SEQ ID NO: 14 - protein, 9 aa, Homo sapiens
  REGION 1..9: note = E07 Light CDR3
QQSYSTLLT

SEQ ID NO: 15 - protein, 11 aa, Homo sapiens
  REGION 1..11: note = C08 Light CDR3
QVWDSSSDHVV

SEQ ID NO: 16 - protein, 10 aa, Homo sapiens
  REGION 1..10: note = G04 Light CDR3
QQSYSTPQVT

SEQ ID NO: 17 - protein, 9 aa, Homo sapiens
  REGION 1..9: note = B07 Light CDR3
QQSYSTPLT

SEQ ID NO: 18 - protein, 9 aa, Homo sapiens
  REGION 1..9: note = C05 Light CDR3
QQFKRYPPT

SEQ ID NO: 19 - protein, 10 aa, Homo sapiens
  REGION 1..10: note = E01 Light CDR3
SSYTSTSTLV

SEQ ID NO: 20 - protein, 9 aa, Homo sapiens
  REGION 1..9: note = E04 Light CDR3
QQSYSTPLT

SEQ ID NO: 21 - protein, 9 aa, Homo sapiens
  REGION 1..9: note = F07 Light CDR3
QQSHSHPPT

SEQ ID NO: 22 - protein, 9 aa, Homo sapiens
  REGION 1..9: note = G06 Light CDR3
QQSYSTPDT

SEQ ID NO: 23 - protein, 9 aa, Homo sapiens
  REGION 1..9: note = G09 Light CDR3
QQSYSTPVT

SEQ ID NO: 24 - protein, 9 aa, Homo sapiens
  REGION 1..9: note = B09 Light CDR3
QQSYSTPLT

SEQ ID NO: 25 - protein, 9 aa, Homo sapiens
  REGION 1..9: note = G10 Light CDR3
QQSYSTLLT

SEQ ID NO: 26 - protein, 8 aa, Homo sapiens
  REGION 1..8: note = E07 Heavy CDR2
ISSSGSTI

SEQ ID NO: 27 - protein, 7 aa, Homo sapiens
  REGION 1..7: note = C08 Heavy CDR2
IYSGGST

SEQ ID NO: 28 - protein, 9 aa, Homo sapiens
  REGION 1..9: note = G04 Heavy CDR2
TYYRSKWST

SEQ ID NO: 29 - protein, 8 aa, Homo sapiens
  REGION 1..8: note = G04 Heavy CDR2
ISSSGSTI

SEQ ID NO: 30 - protein, 8 aa, Homo sapiens
  REGION 1..8: note = C05 Heavy CDR2
ISGGGGTT

SEQ ID NO: 31 - protein, 8 aa, Homo sapiens
  REGION 1..8: note = E01 Heavy CDR2
IYPGDSDT

SEQ ID NO: 32 - protein, 9 aa, Homo sapiens
  REGION 1..9: note = E04 Heavy CDR2
TYYRSKWYN

SEQ ID NO: 33 - protein, 9 aa, Homo sapiens
  REGION 1..9: note = F07 Heavy CDR2
TYYRSKWYN

SEQ ID NO: 34 - protein, 8 aa, Homo sapiens
  REGION 1..8: note = G06 Heavy CDR2
ISSSGSTI

SEQ ID NO: 35 - protein, 9 aa, Homo sapiens
  REGION 1..9: note = G09 Heavy CDR2
TYYGSKWYN

SEQ ID NO: 36 - protein, 8 aa, Homo sapiens
  REGION 1..8: note = B09 Heavy CDR2
ISSSGSTI

SEQ ID NO: 37 - protein, 8 aa, Homo sapiens
  REGION 1..8: note = G10 Heavy CDR2
ISSSGSTI

SEQ ID NO: 38 - protein, 8 aa, Homo sapiens
  REGION 1..8: note = E07 Heavy CDR1
GFTFSDYY

SEQ ID NO: 39 - protein, 8 aa, Homo sapiens
  REGION 1..8: note = C08 Heavy CDR1
GFTVSSNY

SEQ ID NO: 40 - protein, 10 aa, Homo sapiens
  REGION 1..10: note = G04 Heavy CDR1
GDSVSSKSAA

SEQ ID NO: 41 - protein, 8 aa, Homo sapiens
  REGION 1..8: note = B07 Heavy CDR1
GFTFSDYY

SEQ ID NO: 42 - protein, 8 aa, Homo sapiens
  REGION 1..8: note = C05 Heavy CDR1
GFTFSSYA

SEQ ID NO: 43 - protein, 8 aa, Homo sapiens
  REGION 1..8: note = E01 Heavy CDR1
GYSFTSYW

SEQ ID NO: 44 - protein, 10 aa, Homo sapiens
  REGION 1..10: note = E04 Heavy CDR1
GDSVSSNSAA

SEQ ID NO: 45 - protein, 10 aa, Homo sapiens
  REGION 1..10: note = F07 Heavy CDR1
GDSVSSNSAA

SEQ ID NO: 46 - protein, 8 aa, Homo sapiens
  REGION 1..8: note = G06 Heavy CDR1
GFTFSDYY

SEQ ID NO: 47 - protein, 10 aa, Homo sapiens
  REGION 1..10: note = G09 Heavy CDR1
GDSVSSNSAA

SEQ ID NO: 48 - protein, 8 aa, Homo sapiens
  REGION 1..8: note = B09 Heavy CDR1
GFTFSDYY

SEQ ID NO: 49 - protein, 8 aa, Homo sapiens
  REGION 1..8: note = G10 Heavy CDR1
GFTFSDYY

SEQ ID NO: 50 - protein, 6 aa, Homo sapiens
  REGION 1..6: note = E07 Light CDR1
QSIGTY

SEQ ID NO: 51 - protein, 6 aa, Homo sapiens
  REGION 1..6: note = C08 Light CDR1
NIGSQS

SEQ ID NO: 52 - protein, 6 aa, Homo sapiens
  REGION 1..6: note = G04 Light CDR1
QDINDW

SEQ ID NO: 53 - protein, 6 aa, Homo sapiens
  REGION 1..6: note = B07 Light CDR1
QSLSNY

SEQ ID NO: 54 - protein, 6 aa, Homo sapiens
  REGION 1..6: note = C05 Light CDR1
QNIRTW

SEQ ID NO: 55 - protein, 9 aa, Homo sapiens
  REGION 1..9: note = E01 Light CDR1
RSDVGGYNY

SEQ ID NO: 56 - protein, 6 aa, Homo sapiens
  REGION 1..6: note = E04 Light CDR1
QSISTW

SEQ ID NO: 57 - protein, 6 aa, Homo sapiens
  REGION 1..6: note = F07 Light CDR1
QSISSW

SEQ ID NO: 58 - protein, 6 aa, Homo sapiens
  REGION 1..6: note = G06 Light CDR1
QSISSY

SEQ ID NO: 59 - protein, 6 aa, Homo sapiens
  REGION 1..6: note = G09 Light CDR1
QSISTW

SEQ ID NO: 60 - protein, 6 aa, Homo sapiens
  REGION 1..6: note = B09 Light CDR1
QDISNY

SEQ ID NO: 61 - protein, 6 aa, Homo sapiens
  REGION 1..6: note = G10 Light CDR1
QSISSH

SEQ ID NO: 62 - protein, 118 aa, Homo sapiens
  REGION 1..118: note = E07 VH region
QVQLVESGGGLVKPGGSLRLSCAASGFTFSDYYMSWIRQAPGKGLEWVSYISSSGSTIYYADSVKGRFTISRDNAKNSLYLQMNSLRAEDTAVYYCARVDYADAFDIWGQGTLVTVSS

SEQ ID NO: 63 - protein, 117 aa, Homo sapiens
  REGION 1..117: note = C08 VH region
EVQLLESGGGLVQPGRSLRLSCAASGFTVSSNYMSWVRQAPGKGLEWVSVIYSGGSTYYADSVKGRFTISRDNSKNTLYLQMNSLRAEDTAVYYCASPIELGAFDIWGQGTLVTVSS

SEQ ID NO: 64 - protein, 120 aa, Homo sapiens
  REGION 1..120: note = G04 VH region
QVQLQQSGPGLVKPSQTLSLTCAISGDSVSSKSAAWNWIRQSPSRGLEWLGRTYYRSKWSTDYAASVKSRITINPDTSKNQLSLQLNSVTPEDTAVYYCARTWSGYVDVWGQGTLVTVSS

SEQ ID NO: 65 - protein, 118 aa, Homo sapiens
  REGION 1..118: note = B07 VH region
EVQLLESGGGLVKPGGSLRLSCAASGFTFSDYYMSWIRQAPGKGLEWVSYISSSGSTIYYADSVKGRFTISRDNAKNSLYLQMNSLRAEDTAVYYCARENYLNAFDIWGRGTLVTVSS

SEQ ID NO: 66 - protein, 117 aa, Homo sapiens
  REGION 1..117: note = C05 VH region
EVQLLESGGGLVQPGGSLRLSCAASGFTFSSYAMSWVRQAPGKGLEWVSAISGGGGTTYSSDSVKGRFTISRDNSKNTLYLQMNSLRAEDTAVYYCARDSGVAFDIWGQGTLVTVSS

SEQ ID NO: 67 - protein, 119 aa, Homo sapiens
  REGION 1..119: note = E01 VH region
QVQLVQSGAEVKKPGESLKISCKGSGYSFTSYWIGWVRQMPGKGLEWMGIIYPGDSDTRYSPSFQGQVTISADKSISTAYLQWSSLKASDTAMYYCARHQVDTRTADYWGQGTLVTVSS

SEQ ID NO: 68 - protein, 120 aa, Homo sapiens
  REGION 1..120: note = E04 VH region
QVQLQQSGPGLVKPSQTLSLTCAISGDSVSSNSAAWNWIRQSPSRGLEWLGRTYYRSKWYNDYAVSVRSRITINPDTSKNQFSLQLNSVTPEDTAVYYCARSWNDAFDIWGQGTTVTVSS

SEQ ID NO: 69 - protein, 120 aa, Homo sapiens
  REGION 1..120: note = F07 VH region
QVQLQQSGPGLVKPSQTLSLTCVISGDSVSSNSAAWNWIRQSPSRGLEWLGRTYYRSKWYNDYAVSVKSRITINPDTSKNQFSLQLNSVTPEDTAVYYCARDYYYSMDVWGQGTMVTVSS

SEQ ID NO: 70 - protein, 118 aa, Homo sapiens
  REGION 1..118: note = G06 VH region
QVQLVESGGGLVKPGGSLRLSCAASGFTFSDYYMSWIRQAPGKGLEWVSYISSSGSTIYYADSVKGRFTISRDNAKNSLYLQMNSLRAEDTAVYYCARHSWNDAFDVWGQGTLVTVSS

SEQ ID NO: 71 - protein, 120 aa, Homo sapiens
  REGION 1..120: note = G09 VH region
QVQLQQSGPGLVKPSQTLSLTCAISGDSVSSNSAAWNWIRQSPSRGLEWLGRTYYGSKWYNEYALSVKSRIIINPDTSKNQFSLQLNSVTPEDTAVYYCARDYYYSMDVWGQGTLVTVSS

SEQ ID NO: 72 - protein, 118 aa, Homo sapiens
  REGION 1..118: note = B09 VH region
EVQLLESGGGLVKPGGSLRLSCAASGFTFSDYYMSWIRQAPGKGLEWVSYISSSGSTIYYADSVKGRFTISRDNAKNSLYLQMNSLRAEDTAVYYCARHSWSDAFDIWGQGTLVTVSS

SEQ ID NO: 73 - protein, 118 aa, Homo sapiens
  REGION 1..118: note = G10 VH region
EVQLVESGGGLVQPGGSLRLSCAASGFTFSDYYMSWIRQAPGKGLEWVSYISSSGSTIYYADSVKGRFTISRDNAKNSLYLQMNSLRAEDTAVYYCARHSWNDAFDIWGRGTLVTVSS

SEQ ID NO: 74 - protein, 109 aa, Homo sapiens
  REGION 1..109: note = E07 VL region
ASDIQMTQSPSSLSASVGDRVTIACRAGQSIGTYLNWYQQKPGKAPKLLIYVASSLQSGVPSRFSGSGSGTEFTLTISSLQPEDFATYYCQQSYSTLLTFGRGTKVEIK

SEQ ID NO: 75 - protein, 110 aa, Homo sapiens
  REGION 1..110: note = C08 VL region
ASSYELTQPPSVSVAPGKTARITCGGNNIGSQSVHWYQQKPGQAPMLVIYYDSDRPSGIPERFSGSNSGNTATLTISRVEAGDEADYYCQVWDSSSDHVVFGGGTKLTVL

SEQ ID NO: 76 - protein, 110 aa, Homo sapiens
  REGION 1..110: note = G04 VL region
ASDIQMTQSPPALSASVGDRVTITCRASQDINDWLAWYQHKPGKAPKLLIYDASSLESGVPSRFSGSGSGTEFTLTISSLQPDDFATYYCQQSYSTPQVTFGQGTRLEIK

SEQ ID NO: 77 - protein, 109 aa, Homo sapiens
  REGION 1..109: note = B07 VL region
ASDIQMTQSPSSLSASVGDRVTITCRTSQSLSNYLNWYQQKPGKAPKLLIYAASSLQSGVPSRFSGSGSGTDFTLTISSLQPEDFATYYCQQSYSTPLTFGGGTKLEIK

SEQ ID NO: 78 - protein, 109 aa, Homo sapiens
  REGION 1..109: note = C05 VL region
ASDIQMTQSPSFLSASVGDRVTITCRASQNIRTWLAWYQQKPGRAPKLLIYDASSLESGVPSRFSGSGSGTDFTLTISSLQPEDFATYYCQQFKRYPPTFGLGTKVEIK

SEQ ID NO: 79 - protein, 112 aa, Homo sapiens
  REGION 1..112: note = E01 VL region
ASQSALTQPASVSGSPGQSVTISCTGTRSDVGGYNYVSWYQHHPGKAPKLMIYEVSNRPSGVSNRFSGSKSGNTASLTISGLQAEDEADYYCSSYTSTSTLVFGGGTKLTVL

SEQ ID NO: 80 - protein, 109 aa, Homo sapiens
  REGION 1..109: note = E04 VL region
ASDIVMTQSPSTLSASIGDRVTITCRAGQSISTWLAWYQQKPGKAPKLLIYDASSLESGVPLRFSGSGSGTDFTLTISSLQPEDFATYYCQQSYSTPLTFGGGTKVEIK

SEQ ID NO: 81 - protein, 109 aa, Homo sapiens
  REGION 1..109: note = F07 VL region
ASDIQMTQSPSTLSASVGDRVTITCRASQSISSWLAWYQQKPGKAPKLLIYDASSLESGVPLRFSGSGSGTEFTLTISSLQPDDFATYYCQQSHSHPPTFGPGTKVDIK

SEQ ID NO: 82 - protein, 109 aa, Homo sapiens
  REGION 1..109: note = G06 VL region
ASDIQMTQSPSSLSASVGDRVSITCRASQSISSYLNWYQQKPGKAPKLLIYAASSLQSGVPSRFSGSGSGTDFTLTISSLQPEDFATYYCQQSYSTPDTFGGGTKVEIK

SEQ ID NO: 83 - protein, 109 aa, Homo sapiens
  REGION 1..109: note = G09 VL region
ASDIVMTQSPSTLSASIGDRVTITCRAGQSISTWLAWYQQKPGKAPKLLIYDASSLESGVPLRFSGSGSGTEFTLAISSLQPDDFATYYCQQSYSTPVTFGQGTKVEIK

SEQ ID NO: 84 - protein, 109 aa, Homo sapiens
  REGION 1..109: note = B09 VL region
ASDIQMTQSPSSLSASVGDRVTITCQASQDISNYLNWYQQKPGKAPKLLIYDASNLETGVPSRFSGSGSGTDFTLTISSLQPEDFATYYCQQSYSTPLTFGGGTKVEIK

SEQ ID NO: 85 - protein, 109 aa, Homo sapiens
  REGION 1..109: note = G10 VL region
ASDIQMTQSPSSLSASVGDRVTITCRASQSISSHLNWYQQKPGKAPKLLIYAASSLQSGVPSRFSASGSGTDFTLTISSLQPEDFATYYCQQSYSTLLTFGGGTKVEIK

SEQ ID NO: 86 - protein, 240 aa, Homo sapiens
  REGION 1..240: note = E07 scfv
QVQLVESGGGLVKPGGSLRLSCAASGFTFSDYYMSWIRQAPGKGLEWVSYISSSGSTIYYADSVKGRFTISRDNAKNSLYLQMNSLRAEDTAVYYCARVDYADAFDIWGQGTLVTVSSGGGGSGGGGSGGGASDIQMTQSPSSLSASVGDRVTIACRAGQSIGTYLNWYQQKPGKAPKLLIYVASSLQSGVPSRFSGSGSGTEFTLTISSLQPEDFATYYCQQSYSTLLTFGRGTKVEIK

SEQ ID NO: 87 - protein, 240 aa, Homo sapiens
  REGION 1..240: note = C08 scfv
EVQLLESGGGLVQPGRSLRLSCAASGFTVSSNYMSWVRQAPGKGLEWVSVIYSGGSTYYADSVKGRFTISRDNSKNTLYLQMNSLRAEDTAVYYCASPIELGAFDIWGQGTLVTVSSGGGGSGGGGSGGGASSYELTQPPSVSVAPGKTARITCGGNNIGSQSVHWYQQKPGQAPMLVIYYDSDRPSGIPERFSGSNSGNTATLTISRVEAGDEADYYCQVWDSSSDHVVFGGGTKLTVL

SEQ ID NO: 88 - protein, 243 aa, Homo sapiens
  REGION 1..243: note = G04 scfv
QVQLQQSGPGLVKPSQTLSLTCAISGDSVSSKSAAWNWIRQSPSRGLEWLGRTYYRSKWSTDYAASVKSRITINPDTSKNQLSLQLNSVTPEDTAVYYCARTWSGYVDVWGQGTLVTVSSGGGGSGGGGSGGGASDIQMTQSPPALSASVGDRVTITCRASQDINDWLAWYQHKPGKAPKLLIYDASSLESGVPSRFSGSGSGTEFTLTISSLQPDDFATYYCQQSYSTPQVTFGQGTRLEIK

SEQ ID NO: 89 - protein, 240 aa, Homo sapiens
  REGION 1..240: note = B07 scfv
EVQLLESGGGLVKPGGSLRLSCAASGFTFSDYYMSWIRQAPGKGLEWVSYISSSGSTIYYADSVKGRFTISRDNAKNSLYLQMNSLRAEDTAVYYCARENYLNAFDIWGRGTLVTVSSGGGGSGGGGSGGGASDIQMTQSPSSLSASVGDRVTITCRTSQSLSNYLNWYQQKPGKAPKLLIYAASSLQSGVPSRFSGSGSGTDFTLTISSLQPEDFATYYCQQSYSTPLTFGGGTKLEIK

SEQ ID NO: 90 - protein, 239 aa, Homo sapiens
  REGION 1..239: note = C05 scfv
EVQLLESGGGLVQPGGSLRLSCAASGFTFSSYAMSWVRQAPGKGLEWVSAISGGGGTTYSSDSVKGRFTISRDNSKNTLYLQMNSLRAEDTAVYYCARDSGVAFDIWGQGTLVTVSSGGGGSGGGGSGGGASDIQMTQSPSFLSASVGDRVTITCRASQNIRTWLAWYQQKPGRAPKLLIYDASSLESGVPSRFSGSGSGTDFTLTISSLQPEDFATYYCQQFKRYPPTFGLGTKVEIK

SEQ ID NO: 91 - protein, 244 aa, Homo sapiens
  REGION 1..244: note = E01 scfv
QVQLVQSGAEVKKPGESLKISCKGSGYSFTSYWIGWVRQMPGKGLEWMGIIYPGDSDTRYSPSFQGQVTISADKSISTAYLQWSSLKASDTAMYYCARHQVDTRTADYWGQGTLVTVSSGGGGSGGGGSGGGASQSALTQPASVSGSPGQSVTISCTGTRSDVGGYNYVSWYQHHPGKAPKLMIYEVSNRPSGVSNRFSGSKSGNTASLTISGLQAEDEADYYCSSYTSTSTLVFGGGTKLTVL

SEQ ID NO: 92 - protein, 242 aa, Homo sapiens
  REGION 1..242: note = E04 scfv
QVQLQQSGPGLVKPSQTLSLTCAISGDSVSSNSAAWNWIRQSPSRGLEWLGRTYYRSKWYNDYAVSVRSRITINPDTSKNQFSLQLNSVTPEDTAVYYCARSWNDAFDIWGQGTTVTVSSGGGGSGGGGSGGGASDIVMTQSPSTLSASIGDRVTITCRAGQSISTWLAWYQQKPGKAPKLLIYDASSLESGVPLRFSGSGSGTDFTLTISSLQPEDFATYYCQQSYSTPLTFGGGTKVEIK

SEQ ID NO: 93 - protein, 242 aa, Homo sapiens
  REGION 1..242: note = F07 scfv
QVQLQQSGPGLVKPSQTLSLTCVISGDSVSSNSAAWNWIRQSPSRGLEWLGRTYYRSKWYNDYAVSVKSRITINPDTSKNQFSLQLNSVTPEDTAVYYCARDYYYSMDVWGQGTMVTVSSGGGGSGGGGSGGGASDIQMTQSPSTLSASVGDRVTITCRASQSISSWLAWYQQKPGKAPKLLIYDASSLESGVPLRFSGSGSGTEFTLTISSLQPDDFATYYCQQSHSHPPTFGPGTKVDIK

SEQ ID NO: 94 - protein, 240 aa, Homo sapiens
  REGION 1..240: note = G06 scfv
QVQLVESGGGLVKPGGSLRLSCAASGFTFSDYYMSWIRQAPGKGLEWVSYISSSGSTIYYADSVKGRFTISRDNAKNSLYLQMNSLRAEDTAVYYCARHSWNDAFDVWGQGTLVTVSSGGGGSGGGGSGGGASDIQMTQSPSSLSASVGDRVSITCRASQSISSYLNWYQQKPGKAPKLLIYAASSLQSGVPSRFSGSGSGTDFTLTISSLQPEDFATYYCQQSYSTPDTFGGGTKVEIK

SEQ ID NO: 95 - protein, 242 aa, Homo sapiens
  REGION 1..242: note = G09 scfv
QVQLQQSGPGLVKPSQTLSLTCAISGDSVSSNSAAWNWIRQSPSRGLEWLGRTYYGSKWYNEYALSVKSRIIINPDTSKNQFSLQLNSVTPEDTAVYYCARDYYYSMDVWGQGTLVTVSSGGGGSGGGGSGGGASDIVMTQSPSTLSASIGDRVTITCRAGQSISTWLAWYQQKPGKAPKLLIYDASSLESGVPLRFSGSGSGTEFTLAISSLQPDDFATYYCQQSYSTPVTFGQGTKVEIK

SEQ ID NO: 96 - protein, 240 aa, Homo sapiens
  REGION 1..240: note = B09 scfv
EVQLLESGGGLVKPGGSLRLSCAASGFTFSDYYMSWIRQAPGKGLEWVSYISSSGSTIYYADSVKGRFTISRDNAKNSLYLQMNSLRAEDTAVYYCARHSWSDAFDIWGQGTLVTVSSGGGGSGGGGSGGGASDIQMTQSPSSLSASVGDRVTITCQASQDISNYLNWYQQKPGKAPKLLIYDASNLETGVPSRFSGSGSGTDFTLTISSLQPEDFATYYCQQSYSTPLTFGGGTKVEIK

SEQ ID NO: 97 - protein, 240 aa, Homo sapiens
  REGION 1..240: note = G10 scfv
EVQLVESGGGLVQPGGSLRLSCAASGFTFSDYYMSWIRQAPGKGLEWVSYISSSGSTIYYADSVKGRFTISRDNAKNSLYLQMNSLRAEDTAVYYCARHSWNDAFDIWGRGTLVTVSSGGGGSGGGGSGGGASDIQMTQSPSSLSASVGDRVTITCRASQSISSHLNWYQQKPGKAPKLLIYAASSLQSGVPSRFSASGSGTDFTLTISSLQPEDFATYYCQQSYSTLLTFGGGTKVEIK

SEQ ID NO: 98 - protein, 13 aa, synthetic construct
  REGION 1..13: note = Synthetic linker
GGGGSGGGGSGGG

SEQ ID NO: 99 - DNA, 765 bp, Homo sapiens
  misc_feature 1..765: note = E07 nucleotide
  source 1..765: mol_type = genomic DNA
gccatggcccaggtgcagctggtggagtctgggggaggcttggtcaagcctggagggtccctgagactctcctgtgcagcctctggattcaccttcagtgactactacatgagctggatccgccaggctccagggaaggggctggagtgggtttcatacattagtagtagtggtagtaccatatactacgcagactctgtgaagggccgattcaccatctccagggacaacgccaagaactcactgtatctgcaaatgaacagcctgagagccgaggacacggctgtgtattactgtgcaagggtggactacgctgatgcatttgatatctggggccagggcaccctggtcaccgtctcgagtggtggaggcggttcaggcggaggtggctctggcggtggcgctagcgacatccagatgacccagtctccatcctccctgtctgcatctgtaggagacagagtcaccatcgcttgccgggcaggtcagagcattggcacctatttaaattggtatcagcagaaaccagggaaagcccctaaactcctgatctatgttgcatccagtttgcaaagtggggtcccgtcacggttcagtggcagtggatctgggacagaattcactctcaccatcagcagtctgcaacctgaagattttgcaacttactactgtcaacagagttacagtaccctcctcactttcggcagagggaccaaggtggaaatcaaacgtaccgcggccgcatccgcacatcatcatcaccat

SEQ ID NO: 100 - DNA, 768 bp, Homo sapiens
  misc_feature 1..768: note = C08 nucleotide
  source 1..768: mol_type = genomic DNA
gccatggccgaggtgcagctgttggagtctgggggaggcttggtacagcctggcaggtccctgagactctcctgtgcagcctctgggttcaccgtcagtagcaactacatgagctgggtccgccaggctccagggaaggggctggagtgggtctcagttatttatagcggtggtagcacatactacgcagactccgtgaagggccgattcaccatctccagagacaattccaagaacacgctgtatcttcaaatgaacagcctgagagccgaggacacggctgtgtattactgtgcgagccccatagagctgggtgcttttgatatctggggccaaggaaccctggtcaccgtctcgagtggtggaggcggttcaggcggaggtggctctggcggtggcgctagctcctatgagctgactcagccaccctcagtgtcagtggccccaggaaagacggccaggattacctgtgggggaaacaacattggaagtcaaagtgtgcactggtaccagcagaagccaggccaggcccctatgctggtcatctattatgatagcgaccggccctcagggatccctgagcgattctctggctccaactctgggaacacggccaccctgaccatcagcagggtcgaagccggggatgaggccgactattactgtcaggtgtgggatagtagtagtgatcatgtggtattcggcggcgggaccaagctgaccgtcctaggtcagcccgcggccgcatccgcacatcatcatcaccat

SEQ ID NO: 101 - DNA, 774 bp, Homo sapiens
  misc_feature 1..774: note = G04 nucleotide
  source 1..774: mol_type = genomic DNA
gccatggcccaggtacagctgcagcagtcaggtccaggactggtgaagccctcgcagaccctctcactcacctgtgccatctccggggacagtgtctccagcaaaagtgctgcttggaactggatcaggcagtccccatcgagaggccttgagtggctgggaaggacatactacaggtccaagtggtctactgattatgcagcatctgtgaaaagtcgaataaccatcaacccagacacatccaagaaccagctctccctgcagttaaactctgtgactcccgaggacacggctgtgtattactgtgcaagaacgtggagtggttatgtggacgtctggggccaaggaaccctggtcaccgtctcgagtggtggaggcggttcaggcggaggtggctctggcggtggcgctagcgacatccagatgacccagtcccctcccgccctgtctgcatctgtgggagacagagtcaccatcacttgccgggccagtcaagatattaatgactggttggcctggtatcagcataaacctgggaaagcccctaagctcctgatctatgatgcctccagtttggaaagtggggtcccatcaaggttcagcggcagtggatctgggacagaattcactctcaccatcagcagcctgcagcctgatgattttgcaacttactactgtcaacagagttacagtacccctcaggtcacttttggccaggggacacgactggagatcaaacgtaccgcggccgcatccgcacatcatcatcaccat

SEQ ID NO: 102 - DNA, 765 bp, Homo sapiens
  misc_feature 1..765: note = B07 nucleotide
  source 1..765: mol_type = genomic DNA
gccatggccgaggtgcagctgttggagtctgggggaggcttggtcaagcctggagggtccctgagactctcctgtgcggcctctggattcaccttcagtgactactacatgagctggatccgccaggctccagggaaggggctggagtgggtttcatacattagtagtagtggtagtaccatatactacgcagactctgtgaagggccgattcaccatctccagggacaacgccaagaactcactgtatctgcaaatgaacagcctgagagccgaggacacggccgtgtattactgtgcgagagaaaactatctaaatgcttttgatatctggggccgtggcaccctggtcaccgtctcgagtggtggaggcggttcaggcggaggtggctctggcggtggcgctagcgacatccagatgacccagtctccatcctccctgtctgcatctgtaggagacagagtcaccatcacttgccggacaagtcagagccttagtaattacttaaattggtatcagcagaaaccagggaaagcccctaagctcctgatctatgctgcatccagtttgcaaagtggggtcccatcaaggttcagtggcagtggatctgggacagatttcactctcaccatcagcagtctgcaacctgaagattttgcgacttactactgtcaacagagttacagtacccctctcactttcggcggagggaccaagctagagatcaaacgtaccgcggccgcatccgcacatcatcatcaccat

SEQ ID NO: 103 - DNA, 762 bp, Homo sapiens
  misc_feature 1..762: note = C05 nucleotide
  source 1..762: mol_type = genomic DNA
gccatggccgaggtgcagctgttggagtctgggggaggcttggtacagcctggggggtccctgagactctcctgtgcagcctctggattcacctttagcagctatgccatgagctgggtccgccaggctccagggaaggggctggagtgggtctcagctattagtggtggtggtggtaccacatactcctcagactccgtgaagggccggttcaccatctccagagacaattccaagaacacgctgtatctgcaaatgaacagcctgagagccgaggacacggctgtgtattactgtgcgagagattcaggggttgcttttgatatctggggccaaggaaccctggtcaccgtctcgagtggtggaggcggttcaggcggaggtggctctggcggtggcgctagcgacatccagatgacccagtctccatccttcctgtctgcatctgtaggagacagagtcaccatcacttgccgggccagtcagaatatacgtacctggttggcctggtatcagcagaaaccagggagagcccctaagctcctgatctatgatgcctccagtttggaaagtggggtcccatcaaggttcagcggcagtggatctgggactgatttcactctcaccatcagcagcctgcagcctgaagattttgcaacttattactgtcaacagtttaaacgttaccctccgacgtttggcctggggaccaaggtggagatcaaacgtaccgcggccgcatccgcacatcatcatcaccat

SEQ ID NO: 104 - DNA, 780 bp, Homo sapiens
  misc_feature 1..780: note = E01 nucleotide
  source 1..780: mol_type = genomic DNA
gccatggcccaggtccagctggtacagtctggagcagaggtgaaaaagcccggggagtctctgaagatctcctgtaagggttctggatacagctttaccagctactggatcggctgggtgcgccagatgcccgggaaaggcctggagtggatggggatcatctatcctggtgactctgataccagatacagcccgtccttccaaggccaggtcaccatctcagccgacaagtccatcagcaccgcctacctgcagtggagcagcctgaaggcctcggacaccgccatgtattattgtgcgagacatcaggttgatacacggacggctgattactggggccagggaaccctggtcaccgtctcgagtggtggaggcggttcaggcggaggtggctctggcggtggcgctagccagtctgcgctgactcagcctgcctccgtgtctgggtctcctggacagtcggtcaccatctcctgcactggaaccaggagtgacgttggtggttataactatgtctcctggtaccaacaccacccaggcaaagcccccaaactcatgatttatgaggtcagtaatcggccctcaggggtttctaatcgcttctctggctccaagtctggcaacacggcctccctgaccatctctgggctccaggctgaggacgaggctgattattactgcagctcatatacaagcaccagcactctggtattcggcggagggaccaagctgaccgtcctaggtcagcccgcggccgcatccgcacatcatcatcaccat

SEQ ID NO: 105 - DNA, 771 bp, Homo sapiens
  misc_feature 1..771: note = E04 nucleotide
  source 1..771: mol_type = genomic DNA
gccatggcccaggtacagctgcagcagtcaggtccaggactggtgaagccctcgcagaccctctcactcacctgtgccatctccggggacagtgtctctagcaacagtgctgcttggaactggatcaggcagtccccatcgagaggccttgagtggctgggaaggacatactacaggtccaagtggtataatgattatgcagtatctgtgagaagtcgaataaccatcaacccagacacatccaagaaccagttctccctgcagctgaactctgtgactcccgaggacacggctgtgtattactgtgcaagaagctggaatgatgcttttgatatctgggggcaagggaccacggtcaccgtctcgagtggtggaggcggttcaggcggaggtggctctggcggtggcgctagcgatattgtgatgacacagtctccttccaccctgtctgcatctataggagacagagtcaccatcacttgccgggccggtcagagtattagtacctggttggcctggtatcagcagaaaccagggaaagcccctaagctcctgatctatgatgcctccagtttggaaagtggggtcccattaaggttcagcggcagtggatctgggacagatttcactctcaccatcagcagtctgcaacctgaagattttgcaacttactactgtcaacagagttacagtaccccgctcactttcggcggagggaccaaggtggagatcaaacgtaccgcggccgcatccgcacatcatcatcaccat

SEQ ID NO: 106 - DNA, 771 bp, Homo sapiens
  misc_feature 1..771: note = F07 nucleotide
  source 1..771: mol_type = genomic DNA
gccatggcccaggtacagctgcagcagtcaggtccaggcctggtgaagccctcgcagaccctctcactcacctgtgtcatctccggggacagtgtctctagcaacagtgctgcttggaactggatcaggcagtccccatcgcgaggccttgagtggctgggaaggacatactacaggtccaagtggtataatgattatgcagtatctgtgaaaagtcgaataaccatcaacccagacacatccaagaaccagttctccctgcagctgaactctgtgactcccgaggacacggctgtctattattgtgcaagagactactactacagtatggacgtctggggccaagggacaatggtcaccgtctcgagtggtggaggcggttcaggcggaggtggctctggcggtggcgctagcgacatccagatgacccagtctccctccaccctgtctgcatctgtaggagacagagtcaccatcacttgccgggccagtcagagtattagtagctggttggcctggtatcagcagaaaccagggaaagcccctaagctcctgatctatgatgcctccagtttggaaagtggggtcccattaaggttcagcggcagtggatctgggacagaattcactctcaccatcagcagcctgcagcctgatgattttgcaacttattactgtcaacagagtcacagtcacccccctactttcggccctgggaccaaagtggatatcaaacgtaccgcggccgcatccgcacatcatcatcaccat

SEQ ID NO: 107 - DNA, 765 bp, Homo sapiens
  misc_feature 1..765: note = G06 nucleotide
  source 1..765: mol_type = genomic DNA
gccatggcccaggtgcagctggtggagtctgggggaggcttggtcaagcctggagggtccctgagactctcctgtgcagcctctggattcaccttcagtgactactacatgagctggatccgccaggctccagggaaggggctggagtgggtttcatacattagtagtagtggtagtaccatatactacgcagactctgtgaagggccgattcaccatctccagggacaacgccaagaactcactgtatctgcaaatgaacagcctgagagccgaggacacggccgtgtattactgtgcgagacatagctggaatgatgcttttgatgtctggggccagggaaccctggtcaccgtctcgagtggtggaggcggttcaggcggaggtggctctggcggtggcgctagcgacatccagatgacccagtctccatcctccctgtctgcatctgtaggagacagagtctccatcacctgccgggcaagtcagagcattagcagctatttaaattggtatcagcagaaaccagggaaagcccctaagctcctgatctatgctgcatccagtttgcaaagtggggtcccatcaaggttcagtggcagtggatctgggacagatttcactctcaccatcagcagtctgcaacctgaagattttgcaacttactactgtcagcagagttacagtacccccgacactttcggcggagggaccaaggtggaaatcaaacgtaccgcggccgcatccgcacatcatcatcaccat

SEQ ID NO: 108 - DNA, 771 bp, Homo sapiens
  misc_feature 1..771: note = G09 nucleotide
  source 1..771: mol_type = genomic DNA
gccatggcccaggtacagctgcagcagtcaggtccaggactggtgaagccctcgcagaccctctcactcacctgtgccatctccggggacagtgtctctagcaacagtgctgcttggaactggatcaggcagtccccatcgagaggccttgagtggctgggaaggacatactacgggtccaagtggtataatgagtatgcactatctgtgaaaagtcgaataatcatcaacccagacacatccaagaaccagttctccctgcagctgaactctgtgactcccgaggacacggctgtctattattgtgcaagagactactactacagtatggacgtctggggccagggaaccctggtcaccgtctcgagtggtggaggcggttcaggcggaggtggctctggcggtggcgctagcgatattgtgatgactcagtctccttccaccctgtctgcatctataggagacagagtcaccatcacttgccgggccggtcagagtattagtacctggttggcctggtatcagcagaaaccagggaaagcccctaagctcctgatctatgatgcctccagtttggaaagtggggtcccattaaggttcagcggcagtggatctgggacagaattcactctcgccatcagcagcctgcagcctgatgattttgcaacttactactgtcaacagagttacagtaccccggtaacttttggccaggggaccaaggtggagatcaaacgtaccgcggccgcatccgcacatcatcatcaccat

SEQ ID NO: 109 - DNA, 765 bp, Homo sapiens
  misc_feature 1..765: note = B09 nucleotide
  source 1..765: mol_type = genomic DNA
gccatggccgaggtgcagctgttggagtctgggggaggcttggtcaagcctggagggtccctgagactctcctgtgcagcctctggattcaccttcagtgactactacatgagctggatccgccaggctccagggaaggggctggagtgggtttcatacattagtagtagtggtagtaccatatactacgcagactctgtgaagggccgattcaccatctccagggacaacgccaagaactcactgtatctgcaaatgaacagcctgagagccgaggacacggccgtgtattactgtgcgagacatagctggagtgatgcttttgatatctggggccaaggaaccctggtcaccgtctcgagtggtggaggcggttcaggcggaggtggctctggcggtggcgctagcgacatccagatgacccagtctccatcctccctgtctgcatctgtaggagacagagtcaccatcacttgccaggcgagtcaggacattagcaactatttaaattggtatcagcagaaaccagggaaagcccctaagctcctgatctacgatgcatccaatttggaaacaggggtcccatcaaggttcagtggaagtggatctgggacagatttcactctcaccatcagcagtctgcaacctgaagattttgcaacttactactgtcaacagagttacagtactcctctcactttcggcggagggaccaaggtggagatcaaacgtaccgcggccgcatccgcacatcatcatcaccat

SEQ ID NO: 110 - DNA, 765 bp, Homo sapiens
  misc_feature 1..765: note = G10 nucleotide
  source 1..765: mol_type = genomic DNA
gccatggccgaagtgcagctggtggagtccgggggaggcttagttcagcctggggggtccctgagactctcctgtgcagcctctggattcaccttcagtgactactacatgagctggatccgccaggctccagggaaggggctggagtgggtttcatacattagtagtagtggtagtaccatatactacgcagactctgtgaagggccgattcaccatctccagggacaacgccaagaactcactgtatctgcaaatgaacagcctgagagccgaggacacggccgtgtattactgtgcgagacatagctggaatgatgcttttgatatctggggccgtggcaccctggtcaccgtctcgagtggtggaggcggttcaggcggaggtggctctggcggtggcgctagcgacatccagatgacccagtctccatcctccctgtctgcatctgtaggagacagagtcaccatcacttgccgggcaagtcagagcattagcagccatttaaattggtatcagcagaaaccagggaaagcccctaagctcctgatctatgctgcatccagtttgcaaagtggggtcccatccaggttcagtgccagtggatctgggacagatttcactctcaccatcagcagcctgcagcctgaagattttgcaacttactactgtcaacagagttacagtaccctgctcactttcggcggagggaccaaggtggaaatcaaacgtaccgcggccgcatccgcacatcatcatcaccat

SEQ ID NO: 111 - protein, 664 aa, Homo sapiens
  REGION 1..664: note = E07 full heavy and light
ASDIQMTQSPSSLSASVGDRVTIACRAGQSIGTYLNWYQQKPGKAPKLLIYVASSLQSGVPSRFSGSGSGTEFTLTISSLQPEDFATYYCQQSYSTLLTFGRGTKVEIKRTAAAPSVFIFPPSDEQLKSGTASVVCLLNNFYPREAKVQWKVDNALQSGNSQESVTEQDSKDSTYSLSSTLTLSKADYEKHKLYACEVTHQGLSSPVTKSFNRGECQVQLVESGGGLVKPGGSLRLSCAASGFTFSDYYMSWIRQAPGKGLEWVSYISSSGSTIYYADSVKGRFTISRDNAKNSLYLQMNSLRAEDTAVYYCARVDYADAFDIWGQGTLVTVSSASTKGPSVFPLAPSSKSTSGGTAALGCLVKDYFPEPVTVSWNSGALTSGVHTFPAVLQSSGLYSLSSVVTVPSSSLGTQTYICNVNHKPSNTKVDKKVEPKSCDKTHTCPPCPAPELLGGPSVFLFPPKPKDTLMISRTPEVTCVVVDVSHEDPEVKFNWYVDGVEVHNAKTKPREEQYNSTYRVVSVLTVLHQDWLNGKEYKCKVSNKALPAPIEKTISKAKGQPREPQVYTLPPSRDELTKNQVSLTCLVKGFYPSDIAVEWESNGQPENNYKTTPPVLDSDGSFFLYSKLTVDKSRWQQGNVFSCSVMHEALHNHYTQKSLSLSPGK

SEQ ID NO: 112 - protein, 667 aa, Homo sapiens
  REGION 1..667: note = C08 full heavy and light
ASDIQMTQSPPALSASVGDRVTITCRASQDINDWLAWYQHKPGKAPKLLIYDASSLESGVPSRFSGSGSGTEFTLTISSLQPDDFATYYCQQSYSTPQVTFGQGTRLEIKRTAAAPSVFIFPPSDEQLKSGTASVVCLLNNFYPREAKVQWKVDNALQSGNSQESVTEQDSKDSTYSLSSTLTLSKADYEKHKLYACEVTHQGLSSPVTKSFNRGECQVQLQQSGPGLVKPSQTLSLTCAISGDSVSSKSAAWNWIRQSPSRGLEWLGRTYYRSKWSTDYAASVKSRITINPDTSKNQLSLQLNSVTPEDTAVYYCARTWSGYVDVWGQGTLVTVSSASTKGPSVFPLAPSSKSTSGGTAALGCLVKDYFPEPVTVSWNSGALTSGVHTFPAVLQSSGLYSLSSVVTVPSSSLGTQTYICNVNHKPSNTKVDKKVEPKSCDKTHTCPPCPAPELLGGPSVFLFPPKPKDTLMISRTPEVTCVVVDVSHEDPEVKFNWYVDGVEVHNAKTKPREEQYNSTYRVVSVLTVLHQDWLNGKEYKCKVSNKALPAPIEKTISKAKGQPREPQVYTLPPSRDELTKNQVSLTCLVKGFYPSDIAVEWESNGQPENNYKTTPPVLDSDGSFFLYSKLTVDKSRWQQGNVFSCSVMHEALHNHYTQKSLSLSPGK

SEQ ID NO: 113 - protein, 664 aa, Homo sapiens
  REGION 1..664: note = G04 full heavy and light
ASDIQMTQSPSSLSASVGDRVTITCRTSQSLSNYLNWYQQKPGKAPKLLIYAASSLQSGVPSRFSGSGSGTDFTLTISSLQPEDFATYYCQQSYSTPLTFGGGTKLEIKRTAAAPSVFIFPPSDEQLKSGTASVVCLLNNFYPREAKVQWKVDNALQSGNSQESVTEQDSKDSTYSLSSTLTLSKADYEKHKLYACEVTHQGLSSPVTKSFNRGECEVQLLESGGGLVKPGGSLRLSCAASGFTFSDYYMSWIRQAPGKGLEWVSYISSSGSTIYYADSVKGRFTISRDNAKNSLYLQMNSLRAEDTAVYYCARENYLNAFDIWGRGTLVTVSSASTKGPSVFPLAPSSKSTSGGTAALGCLVKDYFPEPVTVSWNSGALTSGVHTFPAVLQSSGLYSLSSVVTVPSSSLGTQTYICNVNHKPSNTKVDKKVEPKSCDKTHTCPPCPAPELLGGPSVFLFPPKPKDTLMISRTPEVTCVVVDVSHEDPEVKFNWYVDGVEVHNAKTKPREEQYNSTYRVVSVLTVLHQDWLNGKEYKCKVSNKALPAPIEKTISKAKGQPREPQVYTLPPSRDELTKNQVSLTCLVKGFYPSDIAVEWESNGQPENNYKTTPPVLDSDGSFFLYSKLTVDKSRWQQGNVFSCSVMHEALHNHYTQKSLSLSPGK

SEQ ID NO: 114 - protein, 663 aa, Homo sapiens
  REGION 1..663: note = B07 full heavy and light
ASDIQMTQSPSFLSASVGDRVTITCRASQNIRTWLAWYQQKPGRAPKLLIYDASSLESGVPSRFSGSGSGTDFTLTISSLQPEDFATYYCQQFKRYPPTFGLGTKVEIKRTAAAPSVFIFPPSDEQLKSGTASVVCLLNNFYPREAKVQWKVDNALQSGNSQESVTEQDSKDSTYSLSSTLTLSKADYEKHKLYACEVTHQGLSSPVTKSFNRGECEVQLLESGGGLVQPGGSLRLSCAASGFTFSSYAMSWVRQAPGKGLEWVSAISGGGGTTYSSDSVKGRFTISRDNSKNTLYLQMNSLRAEDTAVYYCARDSGVAFDIWGQGTLVTVSSASTKGPSVFPLAPSSKSTSGGTAALGCLVKDYFPEPVTVSWNSGALTSGVHTFPAVLQSSGLYSLSSVVTVPSSSLGTQTYICNVNHKPSNTKVDKKVEPKSCDKTHTCPPCPAPELLGGPSVFLFPPKPKDTLMISRTPEVTCVVVDVSHEDPEVKFNWYVDGVEVHNAKTKPREEQYNSTYRVVSVLTVLHQDWLNGKEYKCKVSNKALPAPIEKTISKAKGQPREPQVYTLPPSRDELTKNQVSLTCLVKGFYPSDIAVEWESNGQPENNYKTTPPVLDSDGSFFLYSKLTVDKSRWQQGNVFSCSVMHEALHNHYTQKSLSLSPGK

SEQ ID NO: 115 - protein, 667 aa, Homo sapiens
  REGION 1..667: note = C05 full heavy and light
ASQSALTQPASVSGSPGQSVTISCTGTRSDVGGYNYVSWYQHHPGKAPKLMIYEVSNRPSGVSNRFSGSKSGNTASLTISGLQAEDEADYYCSSYTSTSTLVFGGGTKLTVLGQPAAAPSVTLFPPSSEELQANKATLVCLISDFYPGAVTVAWKADSSPVKAGVETTTPSKQSNNKYAASSYLSLTPEQWKSHRSYSCQVTHEGSTVEKTVAPTECSQVQLVQSGAEVKKPGESLKISCKGSGYSFTSYWIGWVRQMPGKGLEWMGIIYPGDSDTRYSPSFQGQVTISADKSISTAYLQWSSLKASDTAMYYCARHQVDTRTADYWGQGTLVTVSSASTKGPSVFPLAPSSKSTSGGTAALGCLVKDYFPEPVTVSWNSGALTSGVHTFPAVLQSSGLYSLSSVVTVPSSSLGTQTYICNVNHKPSNTKVDKKVEPKSCDKTHTCPPCPAPELLGGPSVFLFPPKPKDTLMISRTPEVTCVVVDVSHEDPEVKFNWYVDGVEVHNAKTKPREEQYNSTYRVVSVLTVLHQDWLNGKEYKCKVSNKALPAPIEKTISKAKGQPREPQVYTLPPSRDELTKNQVSLTCLVKGFYPSDIAVEWESNGQPENNYKTTPPVLDSDGSFFLYSKLTVDKSRWQQGNVFSCSVMHEALHNHYTQKSLSLSPGK

SEQ ID NO: 116 - protein, 663 aa, Homo sapiens
  REGION 1..663: note = E01 full heavy and light
ASSYELTQPPSVSVAPGKTARITCGGNNIGSQSVHWYQQKPGQAPMLVIYYDSDRPSGIPERFSGSNSGNTATLTISRVEAGDEADYYCQVWDSSSDHVVFGGGTKLTVLGQPAAAPSVTLFPPSSEELQANKATLVCLISDFYPGAVTVAWKADSSPVKAGVETTTPSKQSNNKYAASSYLSLTPEQWKSHRSYSCQVTHEGSTVEKTVAPTECSEVQLLESGGGLVQPGRSLRLSCAASGFTVSSNYMSWVRQAPGKGLEWVSVIYSGGSTYYADSVKGRFTISRDNSKNTLYLQMNSLRAEDTAVYYCASPIELGAFDIWGQGTLVTVSSASTKGPSVFPLAPSSKSTSGGTAALGCLVKDYFPEPVTVSWNSGALTSGVHTFPAVLQSSGLYSLSSVVTVPSSSLGTQTYICNVNHKPSNTKVDKKVEPKSCDKTHTCPPCPAPELLGGPSVFLFPPKPKDTLMISRTPEVTCVVVDVSHEDPEVKFNWYVDGVEVHNAKTKPREEQYNSTYRVVSVLTVLHQDWLNGKEYKCKVSNKALPAPIEKTISKAKGQPREPQVYTLPPSRDELTKNQVSLTCLVKGFYPSDIAVEWESNGQPENNYKTTPPVLDSDGSFFLYSKLTVDKSRWQQGNVFSCSVMHEALHNHYTQKSLSLSPGK

SEQ ID NO: 117 - protein, 666 aa, Homo sapiens
  REGION 1..666: note = E04 full heavy and light
ASDIVMTQSPSTLSASIGDRVTITCRAGQSISTWLAWYQQKPGKAPKLLIYDASSLESGVPLRFSGSGSGTDFTLTISSLQPEDFATYYCQQSYSTPLTFGGGTKVEIKRTAAAPSVFIFPPSDEQLKSGTASVVCLLNNFYPREAKVQWKVDNALQSGNSQESVTEQDSKDSTYSLSSTLTLSKADYEKHKLYACEVTHQGLSSPVTKSFNRGECQVQLQQSGPGLVKPSQTLSLTCAISGDSVSSNSAAWNWIRQSPSRGLEWLGRTYYRSKWYNDYAVSVRSRITINPDTSKNQFSLQLNSVTPEDTAVYYCARSWNDAFDIWGQGTTVTVSSASTKGPSVFPLAPSSKSTSGGTAALGCLVKDYFPEPVTVSWNSGALTSGVHTFPAVLQSSGLYSLSSVVTVPSSSLGTQTYICNVNHKPSNTKVDKKVEPKSCDKTHTCPPCPAPELLGGPSVFLFPPKPKDTLMISRTPEVTCVVVDVSHEDPEVKFNWYVDGVEVHNAKTKPREEQYNSTYRVVSVLTVLHQDWLNGKEYKCKVSNKALPAPIEKTISKAKGQPREPQVYTLPPSRDELTKNQVSLTCLVKGFYPSDIAVEWESNGQPENNYKTTPPVLDSDGSFFLYSKLTVDKSRWQQGNVFSCSVMHEALHNHYTQKSLSLSPGK

SEQ ID NO: 118 - protein, 666 aa, Homo sapiens
  REGION 1..666: note = F07 full heavy and light
ASDIQMTQSPSTLSASVGDRVTITCRASQSISSWLAWYQQKPGKAPKLLIYDASSLESGVPLRFSGSGSGTEFTLTISSLQPDDFATYYCQQSHSHPPTFGPGTKVDIKRTAAAPSVFIFPPSDEQLKSGTASVVCLLNNFYPREAKVQWKVDNALQSGNSQESVTEQDSKDSTYSLSSTLTLSKADYEKHKLYACEVTHQGLSSPVTKSFNRGECQVQLQQSGPGLVKPSQTLSLTCVISGDSVSSNSAAWNWIRQSPSRGLEWLGRTYYRSKWYNDYAVSVKSRITINPDTSKNQFSLQLNSVTPEDTAVYYCARDYYYSMDVWGQGTMVTVSSASTKGPSVFPLAPSSKSTSGGTAALGCLVKDYFPEPVTVSWNSGALTSGVHTFPAVLQSSGLYSLSSVVTVPSSSLGTQTYICNVNHKPSNTKVDKKVEPKSCDKTHTCPPCPAPELLGGPSVFLFPPKPKDTLMISRTPEVTCVVVDVSHEDPEVKFNWYVDGVEVHNAKTKPREEQYNSTYRVVSVLTVLHQDWLNGKEYKCKVSNKALPAPIEKTISKAKGQPREPQVYTLPPSRDELTKNQVSLTCLVKGFYPSDIAVEWESNGQPENNYKTTPPVLDSDGSFFLYSKLTVDKSRWQQGNVFSCSVMHEALHNHYTQKSLSLSPGK

SEQ ID NO: 119 - protein, 664 aa, Homo sapiens
  REGION 1..664: note = G06 full heavy and light
ASDIQMTQSPSSLSASVGDRVSITCRASQSISSYLNWYQQKPGKAPKLLIYAASSLQSGVPSRFSGSGSGTDFTLTISSLQPEDFATYYCQQSYSTPDTFGGGTKVEIKRTAAAPSVFIFPPSDEQLKSGTASVVCLLNNFYPREAKVQWKVDNALQSGNSQESVTEQDSKDSTYSLSSTLTLSKADYEKHKLYACEVTHQGLSSPVTKSFNRGECQVQLVESGGGLVKPGGSLRLSCAASGFTFSDYYMSWIRQAPGKGLEWVSYISSSGSTIYYADSVKGRFTISRDNAKNSLYLQMNSLRAEDTAVYYCARHSWNDAFDVWGQGTLVTVSSASTKGPSVFPLAPSSKSTSGGTAALGCLVKDYFPEPVTVSWNSGALTSGVHTFPAVLQSSGLYSLSSVVTVPSSSLGTQTYICNVNHKPSNTKVDKKVEPKSCDKTHTCPPCPAPELLGGPSVFLFPPKPKDTLMISRTPEVTCVVVDVSHEDPEVKFNWYVDGVEVHNAKTKPREEQYNSTYRVVSVLTVLHQDWLNGKEYKCKVSNKALPAPIEKTISKAKGQPREPQVYTLPPSRDELTKNQVSLTCLVKGFYPSDIAVEWESNGQPENNYKTTPPVLDSDGSFFLYSKLTVDKSRWQQGNVFSCSVMHEALHNHYTQKSLSLSPGK

SEQ ID NO: 120 - protein, 666 aa, Homo sapiens
  REGION 1..666: note = G09 full heavy and light
ASDIVMTQSPSTLSASIGDRVTITCRAGQSISTWLAWYQQKPGKAPKLLIYDASSLESGVPLRFSGSGSGTEFTLAISSLQPDDFATYYCQQSYSTPVTFGQGTKVEIKRTAAAPSVFIFPPSDEQLKSGTASVVCLLNNFYPREAKVQWKVDNALQSGNSQESVTEQDSKDSTYSLSSTLTLSKADYEKHKLYACEVTHQGLSSPVTKSFNRGECQVQLQQSGPGLVKPSQTLSLTCAISGDSVSSNSAAWNWIRQSPSRGLEWLGRTYYGSKWYNEYALSVKSRIIINPDTSKNQFSLQLNSVTPEDTAVYYCARDYYYSMDVWGQGTLVTVSSASTKGPSVFPLAPSSKSTSGGTAALGCLVKDYFPEPVTVSWNSGALTSGVHTFPAVLQSSGLYSLSSVVTVPSSSLGTQTYICNVNHKPSNTKVDKKVEPKSCDKTHTCPPCPAPELLGGPSVFLFPPKPKDTLMISRTPEVTCVVVDVSHEDPEVKFNWYVDGVEVHNAKTKPREEQYNSTYRVVSVLTVLHQDWLNGKEYKCKVSNKALPAPIEKTISKAKGQPREPQVYTLPPSRDELTKNQVSLTCLVKGFYPSDIAVEWESNGQPENNYKTTPPVLDSDGSFFLYSKLTVDKSRWQQGNVFSCSVMHEALHNHYTQKSLSLSPGK

SEQ ID NO: 121 - protein, 664 aa, Homo sapiens
  REGION 1..664: note = B09 full heavy and light
ASDIQMTQSPSSLSASVGDRVTITCQASQDISNYLNWYQQKPGKAPKLLIYDASNLETGVPSRFSGSGSGTDFTLTISSLQPEDFATYYCQQSYSTPLTFGGGTKVEIKRTAAAPSVFIFPPSDEQLKSGTASVVCLLNNFYPREAKVQWKVDNALQSGNSQESVTEQDSKDSTYSLSSTLTLSKADYEKHKLYACEVTHQGLSSPVTKSFNRGECEVQLLESGGGLVKPGGSLRLSCAASGFTFSDYYMSWIRQAPGKGLEWVSYISSSGSTIYYADSVKGRFTISRDNAKNSLYLQMNSLRAEDTAVYYCARHSWSDAFDIWGQGTLVTVSSASTKGPSVFPLAPSSKSTSGGTAALGCLVKDYFPEPVTVSWNSGALTSGVHTFPAVLQSSGLYSLSSVVTVPSSSLGTQTYICNVNHKPSNTKVDKKVEPKSCDKTHTCPPCPAPELLGGPSVFLFPPKPKDTLMISRTPEVTCVVVDVSHEDPEVKFNWYVDGVEVHNAKTKPREEQYNSTYRVVSVLTVLHQDWLNGKEYKCKVSNKALPAPIEKTISKAKGQPREPQVYTLPPSRDELTKNQVSLTCLVKGFYPSDIAVEWESNGQPENNYKTTPPVLDSDGSFFLYSKLTVDKSRWQQGNVFSCSVMHEALHNHYTQKSLSLSPGK

SEQ ID NO: 122 - protein, 664 aa, Homo sapiens
  REGION 1..664: note = G10 full heavy and light
ASDIQMTQSPSSLSASVGDRVTITCRASQSISSHLNWYQQKPGKAPKLLIYAASSLQSGVPSRFSASGSGTDFTLTISSLQPEDFATYYCQQSYSTLLTFGGGTKVEIKRTAAAPSVFIFPPSDEQLKSGTASVVCLLNNFYPREAKVQWKVDNALQSGNSQESVTEQDSKDSTYSLSSTLTLSKADYEKHKLYACEVTHQGLSSPVTKSFNRGECEVQLVESGGGLVQPGGSLRLSCAASGFTFSDYYMSWIRQAPGKGLEWVSYISSSGSTIYYADSVKGRFTISRDNAKNSLYLQMNSLRAEDTAVYYCARHSWNDAFDIWGRGTLVTVSSASTKGPSVFPLAPSSKSTSGGTAALGCLVKDYFPEPVTVSWNSGALTSGVHTFPAVLQSSGLYSLSSVVTVPSSSLGTQTYICNVNHKPSNTKVDKKVEPKSCDKTHTCPPCPAPELLGGPSVFLFPPKPKDTLMISRTPEVTCVVVDVSHEDPEVKFNWYVDGVEVHNAKTKPREEQYNSTYRVVSVLTVLHQDWLNGKEYKCKVSNKALPAPIEKTISKAKGQPREPQVYTLPPSRDELTKNQVSLTCLVKGFYPSDIAVEWESNGQPENNYKTTPPVLDSDGSFFLYSKLTVDKSRWQQGNVFSCSVMHEALHNHYTQKSLSLSPGK

SEQ ID NO: 123 - protein, 254 aa, synthetic construct
  REGION 1..254: note = TRDV1(3OMZ) TRAC antigen sequence
AQKVTQAQSSVSMPVRKAVTLNCLYETSWWSYYIFWYKQLPSKEMIFLIRQGSDEQNAKSGRYSVNFKKAAKSVALTISALQLEDSAKYFCALGESLTRADKLIFGKGTRVTVEPNIQNPDPAVYQLRDSKSSDKSVCLFTDFDSQTNVSQSKDSDVYITDKTVLDMRSMDFKSNSAVAWSNKSDFACANAFNNSIIPEDTFFPSPESSCTTAPSAQLKKKLQALKKKNAQLKWKLQALKKKLAQGSGHHHHHH

SEQ ID NO: 124 - protein, 12 aa, synthetic construct
  REGION 1..12: note = Optional scFv tag sequence (kappa sequence + His tag)
RTAAASAHHHHH

SEQ ID NO: 125 - protein, 37 aa, synthetic construct
  REGION 1..37: note = Optional scFv tag sequence (kappa sequence + His and FLAG tag)
RTAAASAHHHHHHKLDYKDHDGDYKDHDIDYKDDDDK

SEQ ID NO: 126 - protein, 13 aa, synthetic construct
  REGION 1..13: note = Optional scFv tag sequence (lambda sequence + His tag)
GQPAAASAHHHHH

SEQ ID NO: 127 - protein, 38 aa, synthetic construct
  REGION 1..38: note = Optional scFv tag sequence (lambda sequence + His and FLAG tag)
GQPAAASAHHHHHHKLDYKDHDGDYKDHDIDYKDDDDK

SEQ ID NO: 128 - protein, 254 aa, Homo sapiens
  REGION 1..254: note = Polymorphic variant of SEQ ID NO: 1
AQKVTQAQSSVSMPVRKAVTLNCLYETSWWSYYIFWYKQLPSKEMIFLIRQGSDEQNAKSGRYSVNFKKAVKSVALTISALQLEDSAKYFCALGESLTRADKLIFGKGTRVTVEPNIQNPDPAVYQLRDSKSSDKSVCLFTDFDSQTNVSQSKDSDVYITDKTVLDMRSMDFKSNSAVAWSNKSDFACANAFNNSIIPEDTFFPSPESSCTTAPSAQLKKKLQALKKKNAQLKWKLQALKKKLAQGSGHHHHHH

SEQ ID NO: 129 - protein, 665 aa, Homo sapiens
  REGION 1..665: note = AD3 (variant 1245_P02_G04 with RTVAAPS sequence instead of RTAAAPS in kappa constant domain)
DIQMTQSPPALSASVGDRVTITCRASQDINDWLAWYQHKPGKAPKLLIYDASSLESGVPSRFSGSGSGTEFTLTISSLQPDDFATYYCQQSYSTPQVTFGQGTRLEIKRTVAAPSVFIFPPSDEQLKSGTASVVCLLNNFYPREAKVQWKVDNALQSGNSQESVTEQDSKDSTYSLSSTLTLSKADYEKHKVYACEVTHQGLSSPVTKSFNRGECEVQLQQSGPGLVKPSQTLSLTCAISGDSVSSKSAAWNWIRQSPSRGLEWLGRTYYRSKWSTDYAASVKSRITINPDTSKNQLSLQLNSVTPEDTAVYYCARTWSGYVDVWGQGTLVTVSSASTKGPSVFPLAPSSKSTSGGTAALGCLVKDYFPEPVTVSWNSGALTSGVHTFPAVLQSSGLYSLSSVVTVPSSSLGTQTYICNVNHKPSNTKVDKKVEPKSCDKTHTCPPCPAPELLGGPSVFLFPPKPKDTLMISRTPEVTCVVVDVSHEDPEVKFNWYVDGVEVHNAKTKPREEQYNSTYRVVSVLTVLHQDWLNGKEYKCKVSNKALPAPIEKTISKAKGQPREPQVYTLPPSRDELTKNQVSLTCLVKGFYPSDIAVEWESNGQPENNYKTTPPVLDSDGSFFLYSKLTVDKSRWQQGNVFSCSVMHEALHNHYTQKSLSLSPGK

SEQ ID NO: 130 - protein, 665 aa, Homo sapiens
  REGION 1..665: note = AD4 (variant 1245_P02_G04 with RTVAAPS sequence instead of RTAAAPS in kappa constant domain)
DIQMTQSPPALSASVGDRVTITCRASQDINDWLAWYQHKPGKAPKLLIYDASSLESGVPSRFSGSGSGTEFTLTISSLQPDDFATYYCQQSYSTPQVTFGQGTRLEIKRTVAAPSVFIFPPSDEQLKSGTASVVCLLNNFYPREAKVQWKVDNALQSGNSQESVTEQDSKDSTYSLSSTLTLSKADYEKHKVYACEVTHQGLSSPVTKSFNRGECEVQLQQSGPGLVKPSQTLSLTCAISGDSVSSKSAAWNWIRQSPSRGLEWLGRTYYRSKWSTDYAASVKSRITINPDTSKNQLSLQLNSVTPEDTAVYYCARTWSGYVDVWGQGTLVTVSSASTKGPSVFPLAPSSKSTSGGTAALGCLVKDYFPEPVTVSWNSGALTSGVHTFPAVLQSSGLYSLSSVVTVPSSSLGTQTYICNVNHKPSNTKVDKKVEPKSCDKTHTCPPCPAPELAGAPSVFLFPPKPKDTLMISRTPEVTCVVVDVSHEDPEVKFNWYVDGVEVHNAKTKPREEQYNSTYRVVSVLTVLHQDWLNGKEYKCKVSNKALPAPIEKTISKAKGQPREPQVYTLPPSRDELTKNQVSLTCLVKGFYPSDIAVEWESNGQPENNYKTTPPVLDSDGSFFLYSKLTVDKSRWQQGNVFSCSVMHEALHNHYTQKSLSLSPGK

SEQ ID NO: 131 - protein, 108 aa, Homo sapiens
  REGION 1..108: note = AD3 and AD4 full light chain variable sequence
DIQMTQSPPALSASVGDRVTITCRASQDINDWLAWYQHKPGKAPKLLIYDASSLESGVPSRFSGSGSGTEFTLTISSLQPDDFATYYCQQSYSTPQVTFGQGTRLEIK

SEQ ID NO: 132 - protein, 120 aa, Homo sapiens
  REGION 1..120: note = AD3 and AD4 full heavy chain variable sequence
EVQLQQSGPGLVKPSQTLSLTCAISGDSVSSKSAAWNWIRQSPSRGLEWLGRTYYRSKWSTDYAASVKSRITINPDTSKNQLSLQLNSVTPEDTAVYYCARTWSGYVDVWGQGTLVTVSS

SEQ ID NO: 133 - protein, 107 aa, Homo sapiens [sequence omitted]

SEQ ID NO: 134 - protein, 330 aa, Homo sapiens [sequence omitted]

SEQ ID NO: 135 - protein, 330 aa, Homo sapiens
  REGION 1..330: note = AD4 full heavy constant domain chain employed (with L235A, G237A modification)
ASTKGPSVFPLAPSSKSTSGGTAALGCLVKDYFPEPVTVSWNSGALTSGVHTFPAVLQSSGLYSLSSVVTVPSSSLGTQTYICNVNHKPSNTKVDKKVEPKSCDKTHTCPPCPAPELAGAPSVFLFPPKPKDTLMISRTPEVTCVVVDVSHEDPEVKFNWYVDGVEVHNAKTKPREEQYNSTYRVVSVLTVLHQDWLNGKEYKCKVSNKALPAPIEKTISKAKGQPREPQVYTLPPSRDELTKNQVSLTCLVKGFYPSDIAVEWESNGQPENNYKTTPPVLDSDGSFFLYSKLTVDKSRWQQGNVFSCSVMHEALHNHYTQKSLSLSPGK

SEQ ID NO: 136 - protein, 667 aa, Homo sapiens
  REGION 1..667: note = 1245_P02_G04 with L235A, G237A) (aka G04 LAGA)
ASDIQMTQSPPALSASVGDRVTITCRASQDINDWLAWYQHKPGKAPKLLIYDASSLESGVPSRFSGSGSGTEFTLTISSLQPDDFATYYCQQSYSTPQVTFGQGTRLEIKRTAAAPSVFIFPPSDEQLKSGTASVVCLLNNFYPREAKVQWKVDNALQSGNSQESVTEQDSKDSTYSLSSTLTLSKADYEKHKLYACEVTHQGLSSPVTKSFNRGECQVQLQQSGPGLVKPSQTLSLTCAISGDSVSSKSAAWNWIRQSPSRGLEWLGRTYYRSKWSTDYAASVKSRITINPDTSKNQLSLQLNSVTPEDTAVYYCARTWSGYVDVWGQGTLVTVSSASTKGPSVFPLAPSSKSTSGGTAALGCLVKDYFPEPVTVSWNSGALTSGVHTFPAVLQSSGLYSLSSVVTVPSSSLGTQTYICNVNHKPSNTKVDKKVEPKSCDKTHTCPPCPAPELAGAPSVFLFPPKPKDTLMISRTPEVTCVVVDVSHEDPEVKFNWYVDGVEVHNAKTKPREEQYNSTYRVVSVLTVLHQDWLNGKEYKCKVSNKALPAPIEKTISKAKGQPREPQVYTLPPSRDELTKNQVSLTCLVKGFYPSDIAVEWESNGQPENNYKTTPPVLDSDGSFFLYSKLTVDKSRWQQGNVFSCSVMHEALHNHYTQKSLSLSPGK

SEQ ID NO: 137 - protein, 664 aa, Homo sapiens
  REGION 1..664: note = 1245_P01_E07 with L235A, G237A (aka E07 LAGA)
ASDIQMTQSPSSLSASVGDRVTIACRAGQSIGTYLNWYQQKPGKAPKLLIYVASSLQSGVPSRFSGSGSGTEFTLTISSLQPEDFATYYCQQSYSTLLTFGRGTKVEIKRTAAAPSVFIFPPSDEQLKSGTASVVCLLNNFYPREAKVQWKVDNALQSGNSQESVTEQDSKDSTYSLSSTLTLSKADYEKHKLYACEVTHQGLSSPVTKSFNRGECQVQLVESGGGLVKPGGSLRLSCAASGFTFSDYYMSWIRQAPGKGLEWVSYISSSGSTIYYADSVKGRFTISRDNAKNSLYLQMNSLRAEDTAVYYCARVDYADAFDIWGQGTLVTVSSASTKGPSVFPLAPSSKSTSGGTAALGCLVKDYFPEPVTVSWNSGALTSGVHTFPAVLQSSGLYSLSSVVTVPSSSLGTQTYICNVNHKPSNTKVDKKVEPKSCDKTHTCPPCPAPELAGAPSVFLFPPKPKDTLMISRTPEVTCVVVDVSHEDPEVKFNWYVDGVEVHNAKTKPREEQYNSTYRVVSVLTVLHQDWLNGKEYKCKVSNKALPAPIEKTISKAKGQPREPQVYTLPPSRDELTKNQVSLTCLVKGFYPSDIAVEWESNGQPENNYKTTPPVLDSDGSFFLYSKLTVDKSRWQQGNVFSCSVMHEALHNHYTQKSLSLSPGK

SEQ ID NO: 138 - protein, 663 aa, Homo sapiens
  REGION 1..663: note = 1252_P01_C08 with L235A, G237A (aka C08 LAGA)
ASSYELTQPPSVSVAPGKTARITCGGNNIGSQSVHWYQQKPGQAPMLVIYYDSDRPSGIPERFSGSNSGNTATLTISRVEAGDEADYYCQVWDSSSDHVVFGGGTKLTVLGQPAAAPSVTLFPPSSEELQANKATLVCLISDFYPGAVTVAWKADSSPVKAGVETTTPSKQSNNKYAASSYLSLTPEQWKSHRSYSCQVTHEGSTVEKTVAPTECSEVQLLESGGGLVQPGRSLRLSCAASGFTVSSNYMSWVRQAPGKGLEWVSVIYSGGSTYYADSVKGRFTISRDNSKNTLYLQMNSLRAEDTAVYYCASPIELGAFDIWGQGTLVTVSSASTKGPSVFPLAPSSKSTSGGTAALGCLVKDYFPEPVTVSWNSGALTSGVHTFPAVLQSSGLYSLSSVVTVPSSSLGTQTYICNVNHKPSNTKVDKKVEPKSCDKTHTCPPCPAPELAGAPSVFLFPPKPKDTLMISRTPEVTCVVVDVSHEDPEVKFNWYVDGVEVHNAKTKPREEQYNSTYRVVSVLTVLHQDWLNGKEYKCKVSNKALPAPIEKTISKAKGQPREPQVYTLPPSRDELTKNQVSLTCLVKGFYPSDIAVEWESNGQPENNYKTTPPVLDSDGSFFLYSKLTVDKSRWQQGNVFSCSVMHEALHNHYTQKSLSLSPGK

SEQ ID NO: 139 - protein, 661 aa, Homo sapiens
  REGION 1..661: note = D1.3 VH/VL + EGFR CH1/CH2/CH3 (LAGA)
ASDIQMTQSPSSLSASVGDRVTITCRASGNIHNYLAWYQQKPGKAPKLLIYYTTTLADGVPSRFSGSGSGTDYTFTISSLQPEDIATYYCQHFWSTPRTFGQGTKVEIKRTAAAPSVFIFPPSDEQLKSGTASVVCLLNNFYPREAKVQWKVDNALQSGNSQESVTEQDSKDSTYSLSSTLTLSKADYEKHKLYACEVTHQGLSSPVTKSFNRGECQVQLQESGPGLVRPSQTLSLTCTVSGSTFSGYGVNWVRQPPGRGLEWIGMIWGDGNTDYNSALKSRVTMLVDTSKNQFSLRLSSVTAADTAVYYCARERDYRLDYWGQGSLVTVSSASTKGPSVFPLAPSSKSTSGGTAALGCLVKDYFPEPVTVSWNSGALTSGVHTFPAVLQSSGLYSLSSVVTVPSSSLGTQTYICNVNHKPSNTKVDKKVEPKSCDKTHTCPPCPAPELAGAPSVFLFPPKPKDTLMISRTPEVTCVVVDVSHEDPEVKFNWYVDGVEVHNAKTKPREEQYNSTYRVVSVLTVLHQDWLNGKEYKCKVSNKALPAPIEKTISKAKGQPREPQVYTLPPSRDETDDGPVSLTCLVKGFYPSDIAVEWESTYGPENNYKTTPPVLDSDGSFFLYSKLTVSYWRWYKGNVFSCSVMHEALHNHYTQKSLSLSPG

SEQ ID NO: 140 - protein, 662 aa, Homo sapiens
  REGION 1..662: note = 1252_P01_C08 VH/VL + CH1/CH2/CH3 EGFR (LAGA)
ASSYELTQPPSVSVAPGKTARITCGGNNIGSQSVHWYQQKPGQAPMLVIYYDSDRPSGIPERFSGSNSGNTATLTISRVEAGDEADYYCQVWDSSSDHVVFGGGTKLTVLGQPAAAPSVTLFPPSSEELQANKATLVCLISDFYPGAVTVAWKADSSPVKAGVETTTPSKQSNNKYAASSYLSLTPEQWKSHRSYSCQVTHEGSTVEKTVAPTECSEVQLLESGGGLVQPGRSLRLSCAASGFTVSSNYMSWVRQAPGKGLEWVSVIYSGGSTYYADSVKGRFTISRDNSKNTLYLQMNSLRAEDTAVYYCASPIELGAFDIWGQGTLVTVSSASTKGPSVFPLAPSSKSTSGGTAALGCLVKDYFPEPVTVSWNSGALTSGVHTFPAVLQSSGLYSLSSVVTVPSSSLGTQTYICNVNHKPSNTKVDKKVEPKSCDKTHTCPPCPAPELAGAPSVFLFPPKPKDTLMISRTPEVTCVVVDVSHEDPEVKFNWYVDGVEVHNAKTKPREEQYNSTYRVVSVLTVLHQDWLNGKEYKCKVSNKALPAPIEKTISKAKGQPREPQVYTLPPSRDETDDGPVSLTCLVKGFYPSDIAVEWESTYGPENNYKTTPPVLDSDGSFFLYSKLTVSYWRWYKGNVFSCSVMHEALHNHYTQKSLSLSPG

SEQ ID NO: 141 - protein, 666 aa, Homo sapiens
  REGION 1..666: note = 1245_P02_G04 VH/VL + CH1/CH2/CH3 EGFR (LAGA)
ASDIQMTQSPPALSASVGDRVTITCRASQDINDWLAWYQHKPGKAPKLLIYDASSLESGVPSRFSGSGSGTEFTLTISSLQPDDFATYYCQQSYSTPQVTFGQGTRLEIKRTAAAPSVFIFPPSDEQLKSGTASVVCLLNNFYPREAKVQWKVDNALQSGNSQESVTEQDSKDSTYSLSSTLTLSKADYEKHKLYACEVTHQGLSSPVTKSFNRGECQVQLQQSGPGLVKPSQTLSLTCAISGDSVSSKSAAWNWIRQSPSRGLEWLGRTYYRSKWSTDYAASVKSRITINPDTSKNQLSLQLNSVTPEDTAVYYCARTWSGYVDVWGQGTLVTVSSASTKGPSVFPLAPSSKSTSGGTAALGCLVKDYFPEPVTVSWNSGALTSGVHTFPAVLQSSGLYSLSSVVTVPSSSLGTQTYICNVNHKPSNTKVDKKVEPKSCDKTHTCPPCPAPELAGAPSVFLFPPKPKDTLMISRTPEVTCVVVDVSHEDPEVKFNWYVDGVEVHNAKTKPREEQYNSTYRVVSVLTVLHQDWLNGKEYKCKVSNKALPAPIEKTISKAKGQPREPQVYTLPPSRDETDDGPVSLTCLVKGFYPSDIAVEWESTYGPENNYKTTPPVLDSDGSFFLYSKLTVSYWRWYKGNVFSCSVMHEALHNHYTQKSLSLSPG

SEQ ID NO: 142 - protein, 663 aa, Homo sapiens
  REGION 1..663: note = 1245_P01_E07 VH/VL + CH1/CH2/CH3 EGFR (LAGA)
ASDIQMTQSPSSLSASVGDRVTIACRAGQSIGTYLNWYQQKPGKAPKLLIYVASSLQSGVPSRFSGSGSGTEFTLTISSLQPEDFATYYCQQSYSTLLTFGRGTKVEIKRTAAAPSVFIFPPSDEQLKSGTASVVCLLNNFYPREAKVQWKVDNALQSGNSQESVTEQDSKDSTYSLSSTLTLSKADYEKHKLYACEVTHQGLSSPVTKSFNRGECQVQLVESGGGLVKPGGSLRLSCAASGFTFSDYYMSWIRQAPGKGLEWVSYISSSGSTIYYADSVKGRFTISRDNAKNSLYLQMNSLRAEDTAVYYCARVDYADAFDIWGQGTLVTVSSASTKGPSVFPLAPSSKSTSGGTAALGCLVKDYFPEPVTVSWNSGALTSGVHTFPAVLQSSGLYSLSSVVTVPSSSLGTQTYICNVNHKPSNTKVDKKVEPKSCDKTHTCPPCPAPELAGAPSVFLFPPKPKDTLMISRTPEVTCVVVDVSHEDPEVKFNWYVDGVEVHNAKTKPREEQYNSTYRVVSVLTVLHQDWLNGKEYKCKVSNKALPAPIEKTISKAKGQPREPQVYTLPPSRDETDDGPVSLTCLVKGFYPSDIAVEWESTYGPENNYKTTPPVLDSDGSFFLYSKLTVSYWRWYKGNVFSCSVMHEALHNHYTQKSLSLSPG

SEQ ID NO: 143 - protein, 917 aa, Homo sapiens
  REGION 1..917: note = D1.3 LAGA + scFV (derived from Cetuximab)
ASDIQMTQSPSSLSASVGDRVTITCRASGNIHNYLAWYQQKPGKAPKLLIYYTTTLADGVPSRFSGSGSGTDYTFTISSLQPEDIATYYCQHFWSTPRTFGQGTKVEIKRTAAAPSVFIFPPSDEQLKSGTASVVCLLNNFYPREAKVQWKVDNALQSGNSQESVTEQDSKDSTYSLSSTLTLSKADYEKHKLYACEVTHQGLSSPVTKSFNRGECQVQLQESGPGLVRPSQTLSLTCTVSGSTFSGYGVNWVRQPPGRGLEWIGMIWGDGNTDYNSALKSRVTMLVDTSKNQFSLRLSSVTAADTAVYYCARERDYRLDYWGQGSLVTVSSASTKGPSVFPLAPSSKSTSGGTAALGCLVKDYFPEPVTVSWNSGALTSGVHTFPAVLQSSGLYSLSSVVTVPSSSLGTQTYICNVNHKPSNTKVDKKVEPKSCDKTHTCPPCPAPELAGAPSVFLFPPKPKDTLMISRTPEVTCVVVDVSHEDPEVKFNWYVDGVEVHNAKTKPREEQYNSTYRVVSVLTVLHQDWLNGKEYKCKVSNKALPAPIEKTISKAKGQPREPQVYTLPPSRDELTKNQVSLTCLVKGFYPSDIAVEWESNGQPENNYKTTPPVLDSDGSFFLYSKLTVDKSRWQQGNVFSCSVMHEALHNHYTQKSLSLSPGGGGGSGGGGSGGGGSQVQLKQSGPGLVQPSQSLSITCTVSGFSLTNYGVHWVRQSPGKGLEWLGVIWSGGNTDYNTPFTSRLSINKDNSKSQVFFKMNSLQSNDTAIYYCARALTYYDYEFAYWGQGTLVTVSAGGGGSGGGGSGGGGSDILLTQSPVILSVSPGERVSFSCRASQSIGTNIHWYQQRTNGSPRLLIKYASESISGIPSRFSGSGSGTDFTLSINSVESEDIADYYCQQNNNWPTTFGAGTKLELK

SEQ ID NO: 144 - protein, 918 aa, Homo sapiens
  REGION 1..918: note = C08 LAGA + scFV (derived from Cetuximab)
ASSYELTQPPSVSVAPGKTARITCGGNNIGSQSVHWYQQKPGQAPMLVIYYDSDRPSGIPERFSGSNSGNTATLTISRVEAGDEADYYCQVWDSSSDHVVFGGGTKLTVLGQPAAAPSVTLFPPSSEELQANKATLVCLISDFYPGAVTVAWKADSSPVKAGVETTTPSKQSNNKYAASSYLSLTPEQWKSHRSYSCQVTHEGSTVEKTVAPTECSEVQLLESGGGLVQPGRSLRLSCAASGFTVSSNYMSWVRQAPGKGLEWVSVIYSGGSTYYADSVKGRFTISRDNSKNTLYLQMNSLRAEDTAVYYCASPIELGAFDIWGQGTLVTVSSASTKGPSVFPLAPSSKSTSGGTAALGCLVKDYFPEPVTVSWNSGALTSGVHTFPAVLQSSGLYSLSSVVTVPSSSLGTQTYICNVNHKPSNTKVDKKVEPKSCDKTHTCPPCPAPELAGAPSVFLFPPKPKDTLMISRTPEVTCVVVDVSHEDPEVKFNWYVDGVEVHNAKTKPREEQYNSTYRVVSVLTVLHQDWLNGKEYKCKVSNKALPAPIEKTISKAKGQPREPQVYTLPPSRDELTKNQVSLTCLVKGFYPSDIAVEWESNGQPENNYKTTPPVLDSDGSFFLYSKLTVDKSRWQQGNVFSCSVMHEALHNHYTQKSLSLSPGGGGGSGGGGSGGGGSQVQLKQSGPGLVQPSQSLSITCTVSGFSLTNYGVHWVRQSPGKGLEWLGVIWSGGNTDYNTPFTSRLSINKDNSKSQVFFKMNSLQSNDTAIYYCARALTYYDYEFAYWGQGTLVTVSAGGGGSGGGGSGGGGSDILLTQSPVILSVSPGERVSFSCRASQSIGTNIHWYQQRTNGSPRLLIKYASESISGIPSRFSGSGSGTDFTLSINSVESEDIADYYCQQNNNWPTTFGAGTKLELK

SEQ ID NO: 145 - protein, 922 aa, Homo sapiens
  REGION 1..922: note = G04 LAGA + scFV (derived from Cetuximab)
ASDIQMTQSPPALSASVGDRVTITCRASQDINDWLAWYQHKPGKAPKLLIYDASSLESGVPSRFSGSGSGTEFTLTISSLQPDDFATYYCQQSYSTPQVTFGQGTRLEIKRTAAAPSVFIFPPSDEQLKSGTASVVCLLNNFYPREAKVQWKVDNALQSGNSQESVTEQDSKDSTYSLSSTLTLSKADYEKHKLYACEVTHQGLSSPVTKSFNRGECQVQLQQSGPGLVKPSQTLSLTCAISGDSVSSKSAAWNWIRQSPSRGLEWLGRTYYRSKWSTDYAASVKSRITINPDTSKNQLSLQLNSVTPEDTAVYYCARTWSGYVDVWGQGTLVTVSSASTKGPSVFPLAPSSKSTSGGTAALGCLVKDYFPEPVTVSWNSGALTSGVHTFPAVLQSSGLYSLSSVVTVPSSSLGTQTYICNVNHKPSNTKVDKKVEPKSCDKTHTCPPCPAPELAGAPSVFLFPPKPKDTLMISRTPEVTCVVVDVSHEDPEVKFNWYVDGVEVHNAKTKPREEQYNSTYRVVSVLTVLHQDWLNGKEYKCKVSNKALPAPIEKTISKAKGQPREPQVYTLPPSRDELTKNQVSLTCLVKGFYPSDIAVEWESNGQPENNYKTTPPVLDSDGSFFLYSKLTVDKSRWQQGNVFSCSVMHEALHNHYTQKSLSLSPGGGGGSGGGGSGGGGSQVQLKQSGPGLVQPSQSLSITCTVSGFSLTNYGVHWVRQSPGKGLEWLGVIWSGGNTDYNTPFTSRLSINKDNSKSQVFFKMNSLQSNDTAIYYCARALTYYDYEFAYWGQGTLVTVSAGGGGSGGGGSGGGGSDILLTQSPVILSVSPGERVSFSCRASQSIGTNIHWYQQRTNGSPRLLIKYASESISGIPSRFSGSGSGTDFTLSINSVESEDIADYYCQQNNNWPTTFGAGTKLELK

SEQ ID NO: 146 - protein, 919 aa, Homo sapiens
  REGION 1..919: note = E07 LAGA + scFV (derived from Cetuximab)
ASDIQMTQSPSSLSASVGDRVTIACRAGQSIGTYLNWYQQKPGKAPKLLIYVASSLQSGVPSRFSGSGSGTEFTLTISSLQPEDFATYYCQQSYSTLLTFGRGTKVEIKRTAAAPSVFIFPPSDEQLKSGTASVVCLLNNFYPREAKVQWKVDNALQSGNSQESVTEQDSKDSTYSLSSTLTLSKADYEKHKLYACEVTHQGLSSPVTKSFNRGECQVQLVESGGGLVKPGGSLRLSCAASGFTFSDYYMSWIRQAPGKGLEWVSYISSSGSTIYYADSVKGRFTISRDNAKNSLYLQMNSLRAEDTAVYYCARVDYADAFDIWGQGTLVTVSSASTKGPSVFPLAPSSKSTSGGTAALGCLVKDYFPEPVTVSWNSGALTSGVHTFPAVLQSSGLYSLSSVVTVPSSSLGTQTYICNVNHKPSNTKVDKKVEPKSCDKTHTCPPCPAPELAGAPSVFLFPPKPKDTLMISRTPEVTCVVVDVSHEDPEVKFNWYVDGVEVHNAKTKPREEQYNSTYRVVSVLTVLHQDWLNGKEYKCKVSNKALPAPIEKTISKAKGQPREPQVYTLPPSRDELTKNQVSLTCLVKGFYPSDIAVEWESNGQPENNYKTTPPVLDSDGSFFLYSKLTVDKSRWQQGNVFSCSVMHEALHNHYTQKSLSLSPGGGGGSGGGGSGGGGSQVQLKQSGPGLVQPSQSLSITCTVSGFSLTNYGVHWVRQSPGKGLEWLGVIWSGGNTDYNTPFTSRLSINKDNSKSQVFFKMNSLQSNDTAIYYCARALTYYDYEFAYWGQGTLVTVSAGGGGSGGGGSGGGGSDILLTQSPVILSVSPGERVSFSCRASQSIGTNIHWYQQRTNGSPRLLIKYASESISGIPSRFSGSGSGTDFTLSINSVESEDIADYYCQQNNNWPTTFGAGTKLELK

SEQ ID NO: 147 - protein, 329 aa, Homo sapiens
  REGION 1..329: note = CH1-CH2-CH3 EGFR binding module
ASTKGPSVFPLAPSSKSTSGGTAALGCLVKDYFPEPVTVSWNSGALTSGVHTFPAVLQSSGLYSLSSVVTVPSSSLGTQTYICNVNHKPSNTKVDKKVEPKSCDKTHTCPPCPAPELLGGPSVFLFPPKPKDTLMISRTPEVTCVVVDVSHEDPEVKFNWYVDGVEVHNAKTKPREEQYNSTYRVVSVLTVLHQDWLNGKEYKCKVSNKALPAPIEKTISKAKGQPREPQVYTLPPSRDETDDGPVSLTCLVKGFYPSDIAVEWESTYGPENNYKTTPPVLDSDGSFFLYSKLTVSYWRWYKGNVFSCSVMHEALHNHYTQKSLSLSPG

SEQ ID NO: 148 - protein, 329 aa, Homo sapiens
  REGION 1..329: note = CH1-CH2-CH3 EGFR binding module (with LAGA)
ASTKGPSVFPLAPSSKSTSGGTAALGCLVKDYFPEPVTVSWNSGALTSGVHTFPAVLQSSGLYSLSSVVTVPSSSLGTQTYICNVNHKPSNTKVDKKVEPKSCDKTHTCPPCPAPELAGAPSVFLFPPKPKDTLMISRTPEVTCVVVDVSHEDPEVKFNWYVDGVEVHNAKTKPREEQYNSTYRVVSVLTVLHQDWLNGKEYKCKVSNKALPAPIEKTISKAKGQPREPQVYTLPPSRDETDDGPVSLTCLVKGFYPSDIAVEWESTYGPENNYKTTPPVLDSDGSFFLYSKLTVSYWRWYKGNVFSCSVMHEALHNHYTQKSLSLSPG

SEQ ID NO: 149 - protein, 241 aa, Homo sapiens
  REGION 1..241: note = scFv (Cetuximab derived) binding module
QVQLKQSGPGLVQPSQSLSITCTVSGFSLTNYGVHWVRQSPGKGLEWLGVIWSGGNTDYNTPFTSRLSINKDNSKSQVFFKMNSLQSNDTAIYYCARALTYYDYEFAYWGQGTLVTVSAGGGGSGGGGSGGGGSDILLTQSPVILSVSPGERVSFSCRASQSIGTNIHWYQQRTNGSPRLLIKYASESISGIPSRFSGSGSGTDFTLSINSVESEDIADYYCQQNNNWPTTFGAGTKLELK

SEQ ID NO: 150 - protein, 20 aa, Homo sapiens
  REGION 1..20: note = N-terminal leader sequence of the V delta 1 chain
MLFSSLLCVFVAFSYSGSSV

SEQ ID NO: 151 - protein, 95 aa, Homo sapiens
  REGION 1..95: note = V region of the V delta 1 chain
AQKVTQAQSSVSMPVRKAVTLNCLYETSWWSYYIFWYKQLPSKEMIFLIRQGSDEQNAKSGRYSVNFKKAAKSVALTISALQLEDSAKYFCALGE

SEQ ID NO: 152 - protein, 16 aa, Homo sapiens
  REGION 1..16: note = J1*0 - one of the four J regions encoded in the human delta one chain germline
TDKLIFGKGTRVTVEP

SEQ ID NO: 153 - protein, 17 aa, Homo sapiens
  REGION 1..17: note = J2*0 - one of the four J regions encoded in the human delta one chain germline
LTAQLFFGKGTQLIVEP

SEQ ID NO: 154 - protein, 19 aa, Homo sapiens
  REGION 1..19: note = J3*0 - one of the four J regions encoded in the human delta one chain germline
SWDTRQMFFGTGIKLFVEP

SEQ ID NO: 155 - protein, 15 aa, Homo sapiens
  REGION 1..15: note = J4*0 - one of the four J regions encoded in the human delta one chain germline
RPLIFGKGTYLEVQQ

SEQ ID NO: 156 - protein, 153 aa, Homo sapiens
  REGION 1..153: note = C1*0 C-region of the V delta 1 chain
  SITE 1: note = Xaa can be any naturally occurring amino acid
XSQPHTKPSVFVMKNGTNVACLVKEFYPKDIRINLVSSKKITEFDPAIVISPSGKYNAVKLGKYESNSVTCSVQHDNKTVHSTDFEVKTDSTDHVKPKETENTKQPSKSCHKPKAIVHTEKVNMMSLTVLGLRMLFAKTVAVNFLLTAKLFFL

SEQ ID NO: 157 - protein, 250 aa, Homo sapiens
  REGION 1..250: note = scFv anti-CD19 binding module
QVQLQQSGAELVRPGSSVKISCKASGYAFSSYWMNWVKQRPGQGLEWIGQIWPGDGDTNYNGKFKGKATLTADESSSTAYMQLSSLASEDSAVYFCARRETTTVGRYYYAMDYWGQGTTVTVSSGGGGSGGGGSGGGGSDIQLTQSPASLAVSLGQRATISCKASQSVDYDGDSYLNWYQQIPGQPPKLLIYDASNLVSGIPPRFSGSGSGTDFTLNIHPVEKVDAATYHCQQSTEDPWTFGGGTKLEIK

SEQ ID NO: 158 - protein, 931 aa, Homo sapiens
  REGION 1..931: note = G04 x Anti-CD19 multispecific (full length)
ASDIQMTQSPPALSASVGDRVTITCRASQDINDWLAWYQHKPGKAPKLLIYDASSLESGVPSRFSGSGSGTEFTLTISSLQPDDFATYYCQQSYSTPQVTFGQGTRLEIKRTAAAPSVFIFPPSDEQLKSGTASVVCLLNNFYPREAKVQWKVDNALQSGNSQESVTEQDSKDSTYSLSSTLTLSKADYEKHKLYACEVTHQGLSSPVTKSFNRGECQVQLQQSGPGLVKPSQTLSLTCAISGDSVSSKSAAWNWIRQSPSRGLEWLGRTYYRSKWSTDYAASVKSRITINPDTSKNQLSLQLNSVTPEDTAVYYCARTWSGYVDVWGQGTLVTVSSASTKGPSVFPLAPSSKSTSGGTAALGCLVKDYFPEPVTVSWNSGALTSGVHTFPAVLQSSGLYSLSSVVTVPSSSLGTQTYICNVNHKPSNTKVDKKVEPKSCDKTHTCPPCPAPELAGAPSVFLFPPKPKDTLMISRTPEVTCVVVDVSHEDPEVKFNWYVDGVEVHNAKTKPREEQYNSTYRVVSVLTVLHQDWLNGKEYKCKVSNKALPAPIEKTISKAKGQPREPQVYTLPPSRDELTKNQVSLTCLVKGFYPSDIAVEWESNGQPENNYKTTPPVLDSDGSFFLYSKLTVDKSRWQQGNVFSCSVMHEALHNHYTQKSLSLSPGGGGGSGGGGSGGGGSQVQLQQSGAELVRPGSSVKISCKASGYAFSSYWMNWVKQRPGQGLEWIGQIWPGDGDTNYNGKFKGKATLTADESSSTAYMQLSSLASEDSAVYFCARRETTTVGRYYYAMDYWGQGTTVTVSSGGGGSGGGGSGGGGSDIQLTQSPASLAVSLGQRATISCKASQSVDYDGDSYLNWYQQIPGQPPKLLIYDASNLVSGIPPRFSGSGSGTDFTLNIHPVEKVDAATYHCQQSTEDPWTFGGGTKLEIK

SEQ ID NO: 159 - protein, 928 aa, Homo sapiens
  REGION 1..928: note = E07 x Anti-CD19 multispecific (full length)
ASDIQMTQSPSSLSASVGDRVTIACRAGQSIGTYLNWYQQKPGKAPKLLIYVASSLQSGVPSRFSGSGSGTEFTLTISSLQPEDFATYYCQQSYSTLLTFGRGTKVEIKRTAAAPSVFIFPPSDEQLKSGTASVVCLLNNFYPREAKVQWKVDNALQSGNSQESVTEQDSKDSTYSLSSTLTLSKADYEKHKLYACEVTHQGLSSPVTKSFNRGECQVQLVESGGGLVKPGGSLRLSCAASGFTFSDYYMSWIRQAPGKGLEWVSYISSSGSTIYYADSVKGRFTISRDNAKNSLYLQMNSLRAEDTAVYYCARVDYADAFDIWGQGTLVTVSSASTKGPSVFPLAPSSKSTSGGTAALGCLVKDYFPEPVTVSWNSGALTSGVHTFPAVLQSSGLYSLSSVVTVPSSSLGTQTYICNVNHKPSNTKVDKKVEPKSCDKTHTCPPCPAPELAGAPSVFLFPPKPKDTLMISRTPEVTCVVVDVSHEDPEVKFNWYVDGVEVHNAKTKPREEQYNSTYRVVSVLTVLHQDWLNGKEYKCKVSNKALPAPIEKTISKAKGQPREPQVYTLPPSRDELTKNQVSLTCLVKGFYPSDIAVEWESNGQPENNYKTTPPVLDSDGSFFLYSKLTVDKSRWQQGNVFSCSVMHEALHNHYTQKSLSLSPGGGGGSGGGGSGGGGSQVQLQQSGAELVRPGSSVKISCKASGYAFSSYWMNWVKQRPGQGLEWIGQIWPGDGDTNYNGKFKGKATLTADESSSTAYMQLSSLASEDSAVYFCARRETTTVGRYYYAMDYWGQGTTVTVSSGGGGSGGGGSGGGGSDIQLTQSPASLAVSLGQRATISCKASQSVDYDGDSYLNWYQQIPGQPPKLLIYDASNLVSGIPPRFSGSGSGTDFTLNIHPVEKVDAATYHCQQSTEDPWTFGGGTKLEIK

SEQ ID NO: 160-171 - skipped (12 entries)

SEQ ID NO: 172 - protein, 92 aa, Homo sapiens
  REGION 1..92: note = Cyno variable delta 1 (V delta 1) chain of a gamma delta T cell receptor (TCR) - aka cyno TRDV1
AQKVTQAQSSVSMPVEKAVTLNCQYETSSWSYDLFWYKQLPGKEMIFLIHQGSSQQNARNGRYSVNFQKAASSITLTISALQLEDSATYFCA

SEQ ID NO: 173 - protein, 101 aa, Homo sapiens
  REGION 1..101: note = Human variable delta 4 chain of a gamma delta T cell receptor (TCR) - aka human TRGV4
KSSNLEGRTKSVIRQTGSSAEITCDLAEGSTGYIHWYLHQEGKAPQRLLYYDSYTSSVVLESGISPGKYDTYGSTRKNLRMILRNLIENDSGVYYCATWDG

SEQ ID NO: 174 - protein, 96 aa, Homo sapiens
  REGION 1..96: note = Human variable delta 2 (V delta 2) chain of a gamma delta T cell receptor (TCR) - aka TRDV2
AIELVPEHQTVPVSIGVPATLRCSMKGEAIGNYYINWYRKTQGNTMTFIYREKDIYGPGFKDNFQGDIDIAKNLAVLKILAPSERDEGSYYCACDT

SEQ ID NO: 175 - protein, 95 aa, Homo sapiens
  REGION 1..95: note = Human variable delta 3 (V delta 3) chain of a gamma delta T cell receptor (TCR) - aka TRDV3
DKVTQSSPDQTVASGSEVVLLCTYDTVYSNPDLFWYRIRPDYSFQFVFYGDNSRSEGADFTQGRFSVKHILTQKAFHLVISPVRTEDSATYYCAF

SEQ ID NO: 176 - protein, 257 aa, Homo sapiens
  REGION 1..257: note = Folate receptor alpha
MAQRMTTQLLLLLVWVAVVGEAQTRIAWARTELLNVCMNAKHHKEKPGPEDKLHEQCRPWRKNACCSTNTSQEAHKDVSYLYRFNWNHCGEMAPACKRHFIQDTCLYECSPNLGPWIQQVDQSWRKERVLNVPLCKEDCEQWWEDCRTSYTCKSNWHKGWNWTSGFNKCAVGAACQPFHFYFPTPTVLCNEIWTHSYKVSNYSRGSGRCIQMWFDPAQGNPNEEVARFYAAAMSGAGPWAAWPFLLSLALMLLWLLS